European Patent Application EP 4 324 920 A1, published February 21, 2024. Title: A method for regulating a gene expression using CRISPR system. Applicant: GenKOre Co., Ltd. Korea Research Institute of Bioscience and Biotechnology. The sequence listing filed with the application follows.

SEQUENCE LISTING (730 sequences)

SEQ ID NO: 1 - RNA, 140 nt, Artificial Sequence
  mature form of Cas12f1 tracrRNA
cuucacugauaaaguggagaaccgcuucaccaaaagcugucccuuaggggauuagaacuugagugaaggugggcugcuugcaucagccuaaugucgagaagugcuuucuucggaaaguaacccucgaaacaaauucauuu

SEQ ID NO: 2 - RNA, 161 nt, Artificial Sequence
  wild-type of Cas12f1 tracrRNA
cuucacugauaaaguggagaaccgcuucaccaaaagcugucccuuaggggauuagaacuugagugaaggugggcugcuugcaucagccuaaugucgagaagugcuuucuucggaaaguaacccucgaaacaaauucauuuuuccucuccaauucugcacaa

SEQ ID NO: 3 - RNA, 17 nt, Artificial Sequence
  mature form of Cas12f1 crRNA repeat
gaaugaaggaaugcaac

SEQ ID NO: 4 - RNA, 37 nt, Artificial Sequence
  wild-type of Cas12f1 crRNA repeat
guugcagaacccgaauagacgaaugaaggaaugcaac

SEQ ID NO: 5 - RNA, 37 nt, Artificial Sequence
  mature form of Cas12f1 crRNA
gaaugaaggaaugcaacnnnnnnnnnnnnnnnnnnnn

SEQ ID NO: 6 - RNA, 57 nt, Artificial Sequence
  wild-type of Cas12f1 crRNA
guugcagaacccgaauagacgaaugaaggaaugcaacnnnnnnnnnnnnnnnnnnnn

SEQ ID NO: 7 - RNA, 161 nt, Artificial Sequence
  mature form of Cas12f1 tracrRNA + GAAA + mature form of Cas12f1 crRNA repeat crRNA repeat
cuucacugauaaaguggagaaccgcuucaccaaaagcugucccuuaggggauuagaacuugagugaaggugggcugcuugcaucagccuaaugucgagaagugcuuucuucggaaaguaacccucgaaacaaauucauuugaaagaaugaaggaaugcaac

SEQ ID NO: 8 - RNA, 181 nt, Artificial Sequence
  mature form of Cas12f1 tracrRNA + GAAA + mature form of Cas12f1 crRNA crRNA
cuucacugauaaaguggagaaccgcuucaccaaaagcugucccuuaggggauuagaacuugagugaaggugggcugcuugcaucagccuaaugucgagaagugcuuucuucggaaaguaacccucgaaacaaauucauuugaaagaaugaaggaaugcaacnnnnnnnnnnnnnnnnnnnn

SEQ ID NO: 9 - RNA, 190 nt, Artificial Sequence
  mature form of Cas12f1 tracrRNA - GAAA - mature form of Cas12f1 crRNA - U-rich tail crRNA - U-rich tail
cuucacugauaaaguggagaaccgcuucaccaaaagcugucccuuaggggauuagaacuugagugaaggugggcugcuugcaucagccuaaugucgagaagugcuuucuucggaaaguaacccucgaaacaaauucauuugaaagaaugaaggaaugcaacnnnnnnnnnnnnnnnnnnnnuuuuauuuu

SEQ ID NO: 10 - RNA, 21 nt, Artificial Sequence
  1st region of Cas12f1 guide RNA
cuucacugauaaaguggagaa

SEQ ID NO: 11 - RNA, 50 nt, Artificial Sequence
  2nd region of Cas12f1 guide RNA
ccgcuucaccaaaagcugucccuuaggggauuagaacuugagugaaggug

SEQ ID NO: 12 - RNA, 56 nt, Artificial Sequence
  3rd region of Cas12f1 guide RNA
ggcugcuugcaucagccuaaugucgagaagugcuuucuucggaaaguaacccucga

SEQ ID NO: 13 - RNA, 13 nt, Artificial Sequence
  4th region of Cas12f1 guide RNA (Mature form)
aacaaauucauuu

SEQ ID NO: 14 - RNA, 34 nt, Artificial Sequence
  4th region of Cas12f1 guide RNA (Wild-type)
aacaaauucauuuuuccucuccaauucugcacaa

SEQ ID NO: 15 - RNA, 10 nt, Artificial Sequence
  5th region of Cas12f1 guide RNA (Mature form)
gaaugaagga

SEQ ID NO: 16 - RNA, 30 nt, Artificial Sequence
  5th region of Cas12f1 guide RNA (Wild-type)
guugcagaacccgaauagacgaaugaagga

SEQ ID NO: 17 - RNA, 10 nt, Artificial Sequence
  first region, 11nt deletion
aaguggagaa

SEQ ID NO: 18 - RNA, 11 nt, Artificial Sequence
  first region, 10nt deletion
aaaguggagaa

SEQ ID NO: 19 - RNA, 12 nt, Artificial Sequence
  first region, 9nt deletion
uaaaguggagaa

SEQ ID NO: 20 - RNA, 13 nt, Artificial Sequence
  first region, 8nt deletion
auaaaguggagaa

SEQ ID NO: 21 - RNA, 14 nt, Artificial Sequence
  first region, 7nt deletion
gauaaaguggagaa

SEQ ID NO: 22 - RNA, 15 nt, Artificial Sequence
  first region, 6nt deletion
ugauaaaguggagaa

SEQ ID NO: 23 - RNA, 16 nt, Artificial Sequence
  first region, 5nt deletion
cugauaaaguggagaa

SEQ ID NO: 24 - RNA, 17 nt, Artificial Sequence
  first region, 4nt deletion
acugauaaaguggagaa

SEQ ID NO: 25 - RNA, 18 nt, Artificial Sequence
  first region, 3nt deletion
cacugauaaaguggagaa

SEQ ID NO: 26 - RNA, 19 nt, Artificial Sequence
  first region, 2nt deletion
ucacugauaaaguggagaa

SEQ ID NO: 27 - RNA, 20 nt, Artificial Sequence
  first region, 1nt deletion
uucacugauaaaguggagaa

SEQ ID NO: 28 - RNA, 10 nt, Artificial Sequence
  deleted part of the first region, 10nt
aaaguggaga

SEQ ID NO: 29 - RNA, 11 nt, Artificial Sequence
  deleted part of the first region, 11nt
uaaaguggaga

SEQ ID NO: 30 - RNA, 12 nt, Artificial Sequence
  deleted part of the first region, 12nt
auaaaguggaga

SEQ ID NO: 31 - RNA, 13 nt, Artificial Sequence
  deleted part of the first region, 13nt
gauaaaguggaga

SEQ ID NO: 32 - RNA, 14 nt, Artificial Sequence
  deleted part of the first region, 14nt
ugauaaaguggaga

SEQ ID NO: 33 - RNA, 15 nt, Artificial Sequence
  deleted part of the first region, 15nt
cugauaaaguggaga

SEQ ID NO: 34 - RNA, 16 nt, Artificial Sequence
  deleted part of the first region, 16nt
acugauaaaguggaga

SEQ ID NO: 35 - RNA, 17 nt, Artificial Sequence
  deleted part of the first region, 17nt
cacugauaaaguggaga

SEQ ID NO: 36 - RNA, 18 nt, Artificial Sequence
  deleted part of the first region, 18nt
ucacugauaaaguggaga

SEQ ID NO: 37 - RNA, 19 nt, Artificial Sequence
  deleted part of the first region, 19nt
uucacugauaaaguggaga

SEQ ID NO: 38 - RNA, 20 nt, Artificial Sequence
  deleted part of the first region, 20nt
cuucacugauaaaguggaga

SEQ ID NO: 39 - RNA, 28 nt, Artificial Sequence
  second region, 11bp deletion
ccgcuucaccauuagugagugaaggugg

SEQ ID NO: 40 - RNA, 30 nt, Artificial Sequence
  second region, 10bp deletion
ccgcuucaccaauuaguugagugaaggugg

SEQ ID NO: 41 - RNA, 32 nt, Artificial Sequence
  second region, 9bp deletion
ccgcuucaccaaauuagcuugagugaaggugg

SEQ ID NO: 42 - RNA, 34 nt, Artificial Sequence
  second region, 8bp deletion
ccgcuucaccaaaauuagacuugagugaaggugg

SEQ ID NO: 43 - RNA, 36 nt, Artificial Sequence
  second region, 7bp deletion
ccgcuucaccaaaaguuagaacuugagugaaggugg

SEQ ID NO: 44 - RNA, 38 nt, Artificial Sequence
  second region, 6bp deletion
ccgcuucaccaaaagcuuaggaacuugagugaaggugg

SEQ ID NO: 45 - RNA, 40 nt, Artificial Sequence
  second region, 5bp deletion
ccgcuucaccaaaagcuuuagagaacuugagugaaggugg

SEQ ID NO: 46 - RNA, 43 nt, Artificial Sequence
  second region, 4bp deletion
ccgcuucaccaaaagcuguuaguuagaacuugagugaaggugg

SEQ ID NO: 47 - RNA, 42 nt, Artificial Sequence
  second region, 4bp+1nt deletion
ccgcuucaccaaaagcuguuaguagaacuugagugaaggugg

SEQ ID NO: 48 - RNA, 45 nt, Artificial Sequence
  second region, 3bp deletion
ccgcuucaccaaaagcuguuuagauuagaacuugagugaaggugg

SEQ ID NO: 49 - RNA, 47 nt, Artificial Sequence
  second region, 2bp deletion
ccgcuucaccaaaagcugucuuaggauuagaacuugagugaaggugg

SEQ ID NO: 50 - RNA, 49 nt, Artificial Sequence
  second region, 1bp deletion
ccgcuucaccaaaagcuguccuuagggauuagaacuugagugaaggugg

SEQ ID NO: 51 - RNA, 11 nt, Artificial Sequence
  second region, 5' remains
ccgcuucacca

SEQ ID NO: 52 - RNA, 13 nt, Artificial Sequence
  second region, 3' remains
ugagugaaggugg

SEQ ID NO: 53 - RNA, 10 nt, Artificial Sequence
  upper-deleted part of the second region, 10nt
aaagcugucc

SEQ ID NO: 54 - RNA, 11 nt, Artificial Sequence
  upper-deleted part of the second region, 11nt
aaagcuguccc

SEQ ID NO: 55 - RNA, 10 nt, Artificial Sequence
  lower-deleted part of the second region, 10nt
gauuagaacu

SEQ ID NO: 56 - RNA, 11 nt, Artificial Sequence
  lower-deleted part of the second region, 11nt
ggauuagaacu

SEQ ID NO: 57 - RNA, 12 nt, Artificial Sequence
  lower-deleted part of the second region, 12nt
gggauuagaacu

SEQ ID NO: 58 - RNA, 10 nt, Artificial Sequence
  intermediate sequence of the second region, 10nt
aaauuagacu

SEQ ID NO: 59 - RNA, 12 nt, Artificial Sequence
  intermediate sequence of the second region, 11nt
aaaguuagaacu

SEQ ID NO: 60 - RNA, 14 nt, Artificial Sequence
  intermediate sequence of the second region, 12nt
aaagcuuaggaacu

SEQ ID NO: 61 - RNA, 16 nt, Artificial Sequence
  intermediate sequence of the second region, 13nt
aaagcuuuagagaacu

SEQ ID NO: 62 - RNA, 18 nt, Artificial Sequence
  intermediate sequence of the second region, 14nt
aaagcuguuaguagaacu

SEQ ID NO: 63 - RNA, 19 nt, Artificial Sequence
  intermediate sequence of the second region, 15nt
aaagcuguuaguuagaacu

SEQ ID NO: 64 - RNA, 21 nt, Artificial Sequence
  intermediate sequence of the second region, 16nt
aaagcuguuuagauuagaacu

SEQ ID NO: 65 - RNA, 23 nt, Artificial Sequence
  intermediate sequence of the second region, 17nt
aaagcugucuuaggauuagaacu

SEQ ID NO: 66 - RNA, 25 nt, Artificial Sequence
  intermediate sequence of the second region, 18nt
aaagcuguccuuagggauuagaacu

SEQ ID NO: 67 - RNA, 10 nt, Artificial Sequence
  fourth region of the tracrRNA(mature form), delete 3nt
aacaaauuca

SEQ ID NO: 68 - RNA, 11 nt, Artificial Sequence
  fourth region of the tracrRNA(mature form), delete 4nt
aacaaauucau

SEQ ID NO: 69 - RNA, 12 nt, Artificial Sequence
  fourth region of the tracrRNA(mature form), delete 5nt
aacaaauucauu

SEQ ID NO: 70 - RNA, 13 nt, Artificial Sequence
  fourth region of the tracrRNA(wild-type), 21nt deletion
aacaaauucauuu

SEQ ID NO: 71 - RNA, 14 nt, Artificial Sequence
  fourth region of the tracrRNA(wild-type), 20nt deletion
aacaaauucauuuu

SEQ ID NO: 72 - RNA, 15 nt, Artificial Sequence
  fourth region of the tracrRNA(wild-type), 19nt deletion
aacaaauucauuuuu

SEQ ID NO: 73 - RNA, 16 nt, Artificial Sequence
  fourth region of the tracrRNA(wild-type), 18nt deletion
aacaaauucauuuuuc

SEQ ID NO: 74 - RNA, 17 nt, Artificial Sequence
  fourth region of the tracrRNA(wild-type), 17nt deletion
aacaaauucauuuuucc

SEQ ID NO: 75 - RNA, 18 nt, Artificial Sequence
  fourth region of the tracrRNA(wild-type), 16nt deletion
aacaaauucauuuuuccu

SEQ ID NO: 76 - RNA, 19 nt, Artificial Sequence
  fourth region of the tracrRNA(wild-type), 15nt deletion
aacaaauucauuuuuccuc

SEQ ID NO: 77 - RNA, 20 nt, Artificial Sequence
  fourth region of the tracrRNA(wild-type), 14nt deletion
aacaaauucauuuuuccucu

SEQ ID NO: 78 - RNA, 21 nt, Artificial Sequence
  fourth region of the tracrRNA(wild-type), 13nt deletion
aacaaauucauuuuuccucuc

SEQ ID NO: 79 - RNA, 22 nt, Artificial Sequence
  fourth region of the tracrRNA(wild-type), 12nt deletion
aacaaauucauuuuuccucucc

SEQ ID NO: 80 - RNA, 23 nt, Artificial Sequence
  fourth region of the tracrRNA(wild-type), 11nt deletion
aacaaauucauuuuuccucucca

SEQ ID NO: 81 - RNA, 24 nt, Artificial Sequence
  fourth region of the tracrRNA(wild-type), 10nt deletion
aacaaauucauuuuuccucuccaa

SEQ ID NO: 82 - RNA, 25 nt, Artificial Sequence
  fourth region of the tracrRNA(wild-type), 9nt deletion
aacaaauucauuuuuccucuccaau

SEQ ID NO: 83 - RNA, 26 nt, Artificial Sequence
  fourth region of the tracrRNA(wild-type), 8nt deletion
aacaaauucauuuuuccucuccaauu

SEQ ID NO: 84 - RNA, 27 nt, Artificial Sequence
  fourth region of the tracrRNA(wild-type), 7nt deletion
aacaaauucauuuuuccucuccaauuc

SEQ ID NO: 85 - RNA, 28 nt, Artificial Sequence
  fourth region of the tracrRNA(wild-type), 6nt deletion
aacaaauucauuuuuccucuccaauucu

SEQ ID NO: 86 - RNA, 29 nt, Artificial Sequence
  fourth region of the tracrRNA(wild-type), 5nt deletion
aacaaauucauuuuuccucuccaauucug

SEQ ID NO: 87 - RNA, 30 nt, Artificial Sequence
  fourth region of the tracrRNA(wild-type), 4nt deletion
aacaaauucauuuuuccucuccaauucugc

SEQ ID NO: 88 - RNA, 31 nt, Artificial Sequence
  fourth region of the tracrRNA(wild-type), 3nt deletion
aacaaauucauuuuuccucuccaauucugca

SEQ ID NO: 89 - RNA, 32 nt, Artificial Sequence
  fourth region of the tracrRNA(wild-type), 2nt deletion
aacaaauucauuuuuccucuccaauucugcac

SEQ ID NO: 90 - RNA, 33 nt, Artificial Sequence
  fourth region of the tracrRNA(wild-type), 1nt deletion
aacaaauucauuuuuccucuccaauucugcaca

SEQ ID NO: 91 - RNA, 10 nt, Artificial Sequence
  fifth region of the crRNA(wild-type), 20nt deletion
gaaugaagga

SEQ ID NO: 92 - RNA, 11 nt, Artificial Sequence
  fifth region of the crRNA(wild-type), 19nt deletion
cgaaugaagga

SEQ ID NO: 93 - RNA, 12 nt, Artificial Sequence
  fifth region of the crRNA(wild-type), 18nt deletion
acgaaugaagga

SEQ ID NO: 94 - RNA, 13 nt, Artificial Sequence
  fifth region of the crRNA(wild-type), 17nt deletion
gacgaaugaagga

SEQ ID NO: 95 - RNA, 14 nt, Artificial Sequence
  fifth region of the crRNA(wild-type), 16nt deletion
agacgaaugaagga

SEQ ID NO: 96 - RNA, 15 nt, Artificial Sequence
  fifth region of the crRNA(wild-type), 15nt deletion
uagacgaaugaagga

SEQ ID NO: 97 - RNA, 16 nt, Artificial Sequence
  fifth region of the crRNA(wild-type), 14nt deletion
auagacgaaugaagga

SEQ ID NO: 98 - RNA, 17 nt, Artificial Sequence
  fifth region of the crRNA(wild-type), 13nt deletion
aauagacgaaugaagga

SEQ ID NO: 99 - RNA, 18 nt, Artificial Sequence
  fifth region of the crRNA(wild-type), 12nt deletion
gaauagacgaaugaagga

SEQ ID NO: 100 - RNA, 19 nt, Artificial Sequence
  fifth region of the crRNA(wild-type), 11nt deletion
cgaauagacgaaugaagga

SEQ ID NO: 101 - RNA, 20 nt, Artificial Sequence
  fifth region of the crRNA(wild-type), 10nt deletion
ccgaauagacgaaugaagga

SEQ ID NO: 102 - RNA, 21 nt, Artificial Sequence
  fifth region of the crRNA(wild-type), 9nt deletion
cccgaauagacgaaugaagga

SEQ ID NO: 103 - RNA, 22 nt, Artificial Sequence
  fifth region of the crRNA(wild-type), 8nt deletion
acccgaauagacgaaugaagga

SEQ ID NO: 104 - RNA, 23 nt, Artificial Sequence
  fifth region of the crRNA(wild-type), 7nt deletion
aacccgaauagacgaaugaagga

SEQ ID NO: 105 - RNA, 24 nt, Artificial Sequence
  fifth region of the crRNA(wild-type), 6nt deletion
gaacccgaauagacgaaugaagga

SEQ ID NO: 106 - RNA, 25 nt, Artificial Sequence
  fifth region of the crRNA(wild-type), 5nt deletion
agaacccgaauagacgaaugaagga

SEQ ID NO: 107 - RNA, 26 nt, Artificial Sequence
  fifth region of the crRNA(wild-type), 4nt deletion
cagaacccgaauagacgaaugaagga

SEQ ID NO: 108 - RNA, 27 nt, Artificial Sequence
  fifth region of the crRNA(wild-type), 3nt deletion
gcagaacccgaauagacgaaugaagga

SEQ ID NO: 109 - RNA, 28 nt, Artificial Sequence
  fifth region of the crRNA(wild-type), 2nt deletion
ugcagaacccgaauagacgaaugaagga

SEQ ID NO: 110 - RNA, 29 nt, Artificial Sequence
  fifth region of the crRNA(wild-type), 1nt deletion
uugcagaacccgaauagacgaaugaagga

SEQ ID NO: 111 - RNA, 13 nt, Artificial Sequence
  fourth region + Linker + fifth region, 7bp deletion (mature form)
aacaaagaaagga

SEQ ID NO: 112 - RNA, 15 nt, Artificial Sequence
  fourth region + Linker + fifth region, 6bp deletion (mature form)
aacaaaugaaaagga

SEQ ID NO: 113 - RNA, 17 nt, Artificial Sequence
  fourth region + Linker + fifth region, 5bp deletion (mature form)
aacaaauugaaaaagga

SEQ ID NO: 114 - RNA, 19 nt, Artificial Sequence
  fourth region + Linker + fifth region, 4bp deletion (mature form)
aacaaauucgaaagaagga

SEQ ID NO: 115 - RNA, 21 nt, Artificial Sequence
  fourth region + Linker + fifth region, 3bp deletion (mature form)
aacaaauucagaaaugaagga

SEQ ID NO: 116 - RNA, 23 nt, Artificial Sequence
  fourth region + Linker + fifth region, 2bp deletion (mature form)
aacaaauucaugaaaaugaagga

SEQ ID NO: 117 - RNA, 25 nt, Artificial Sequence
  fourth region + Linker + fifth region, 1bp deletion (mature form)
aacaaauucauugaaaaaugaagga

SEQ ID NO: 118 - RNA, 27 nt, Artificial Sequence
  fourth region + Linker + fifth region (mature form)
aacaaauucauuugaaagaaugaagga

SEQ ID NO: 119 - RNA, 120 nt, Artificial Sequence
  engineered tracrRNA(mature form, 20nt deletion in the first region)
accgcuucaccaaaagcugucccuuaggggauuagaacuugagugaaggugggcugcuugcaucagccuaaugucgagaagugcuuucuucggaaaguaacccucgaaacaaauucauuu

SEQ ID NO: 120 - RNA, 121 nt, Artificial Sequence
  engineered tracrRNA(mature form, 19nt deletion in the first region)
aaccgcuucaccaaaagcugucccuuaggggauuagaacuugagugaaggugggcugcuugcaucagccuaaugucgagaagugcuuucuucggaaaguaacccucgaaacaaauucauuu

SEQ ID NO: 121 - RNA, 122 nt, Artificial Sequence
  engineered tracrRNA(mature form, 18nt deletion in the first region)
gaaccgcuucaccaaaagcugucccuuaggggauuagaacuugagugaaggugggcugcuugcaucagccuaaugucgagaagugcuuucuucggaaaguaacccucgaaacaaauucauuu

SEQ ID NO: 122 - RNA, 123 nt, Artificial Sequence
  engineered tracrRNA(mature form, 17nt deletion in the first region)
agaaccgcuucaccaaaagcugucccuuaggggauuagaacuugagugaaggugggcugcuugcaucagccuaaugucgagaagugcuuucuucggaaaguaacccucgaaacaaauucauuu

SEQ ID NO: 123 - RNA, 124 nt, Artificial Sequence
  engineered tracrRNA(mature form, 16nt deletion in the first region)
gagaaccgcuucaccaaaagcugucccuuaggggauuagaacuugagugaaggugggcugcuugcaucagccuaaugucgagaagugcuuucuucggaaaguaacccucgaaacaaauucauuu

SEQ ID NO: 124 - RNA, 125 nt, Artificial Sequence
  engineered tracrRNA(mature form, 15nt deletion in the first region)
ggagaaccgcuucaccaaaagcugucccuuaggggauuagaacuugagugaaggugggcugcuugcaucagccuaaugucgagaagugcuuucuucggaaaguaacccucgaaacaaauucauuu

SEQ ID NO: 125 - RNA, 126 nt, Artificial Sequence
  engineered tracrRNA(mature form, 14nt deletion in the first region)
uggagaaccgcuucaccaaaagcugucccuuaggggauuagaacuugagugaaggugggcugcuugcaucagccuaaugucgagaagugcuuucuucggaaaguaacccucgaaacaaauucauuu

SEQ ID NO: 126 - RNA, 127 nt, Artificial Sequence
  engineered tracrRNA(mature form, 13nt deletion in the first region)
guggagaaccgcuucaccaaaagcugucccuuaggggauuagaacuugagugaaggugggcugcuugcaucagccuaaugucgagaagugcuuucuucggaaaguaacccucgaaacaaauucauuu

SEQ ID NO: 127 - RNA, 128 nt, Artificial Sequence
  engineered tracrRNA(mature form, 12nt deletion in the first region)
aguggagaaccgcuucaccaaaagcugucccuuaggggauuagaacuugagugaaggugggcugcuugcaucagccuaaugucgagaagugcuuucuucggaaaguaacccucgaaacaaauucauuu

SEQ ID NO: 128 - RNA, 129 nt, Artificial Sequence
  engineered tracrRNA(mature form, 11nt deletion in the first region)
aaguggagaaccgcuucaccaaaagcugucccuuaggggauuagaacuugagugaaggugggcugcuugcaucagccuaaugucgagaagugcuuucuucggaaaguaacccucgaaacaaauucauuu

SEQ ID NO: 129 - RNA, 130 nt, Artificial Sequence
  engineered tracrRNA(mature form, 10nt deletion in the first region)
aaaguggagaaccgcuucaccaaaagcugucccuuaggggauuagaacuugagugaaggugggcugcuugcaucagccuaaugucgagaagugcuuucuucggaaaguaacccucgaaacaaauucauuu

SEQ ID NO: 130 - RNA, 131 nt, Artificial Sequence
  engineered tracrRNA(mature form, 9nt deletion in the first region)
uaaaguggagaaccgcuucaccaaaagcugucccuuaggggauuagaacuugagugaaggugggcugcuugcaucagccuaaugucgagaagugcuuucuucggaaaguaacccucgaaacaaauucauuu

SEQ ID NO: 131 - RNA, 132 nt, Artificial Sequence
  engineered tracrRNA(mature form, 8nt deletion in the first region)
auaaaguggagaaccgcuucaccaaaagcugucccuuaggggauuagaacuugagugaaggugggcugcuugcaucagccuaaugucgagaagugcuuucuucggaaaguaacccucgaaacaaauucauuu

SEQ ID NO: 132 - RNA, 133 nt, Artificial Sequence
  engineered tracrRNA(mature form, 7nt deletion in the first region)
gauaaaguggagaaccgcuucaccaaaagcugucccuuaggggauuagaacuugagugaaggugggcugcuugcaucagccuaaugucgagaagugcuuucuucggaaaguaacccucgaaacaaauucauuu

SEQ ID NO: 133 - RNA, 134 nt, Artificial Sequence
  engineered tracrRNA(mature form, 6nt deletion in the first region)
ugauaaaguggagaaccgcuucaccaaaagcugucccuuaggggauuagaacuugagugaaggugggcugcuugcaucagccuaaugucgagaagugcuuucuucggaaaguaacccucgaaacaaauucauuu

SEQ ID NO: 134 - RNA, 135 nt, Artificial Sequence
  engineered tracrRNA(mature form, 5nt deletion in the first region)
cugauaaaguggagaaccgcuucaccaaaagcugucccuuaggggauuagaacuugagugaaggugggcugcuugcaucagccuaaugucgagaagugcuuucuucggaaaguaacccucgaaacaaauucauuu

SEQ ID NO: 135 - RNA, 136 nt, Artificial Sequence
  engineered tracrRNA(mature form, 4nt deletion in the first region)
acugauaaaguggagaaccgcuucaccaaaagcugucccuuaggggauuagaacuugagugaaggugggcugcuugcaucagccuaaugucgagaagugcuuucuucggaaaguaacccucgaaacaaauucauuu

SEQ ID NO: 136 - RNA, 137 nt, Artificial Sequence
  engineered tracrRNA(mature form, 3nt deletion in the first region)
cacugauaaaguggagaaccgcuucaccaaaagcugucccuuaggggauuagaacuugagugaaggugggcugcuugcaucagccuaaugucgagaagugcuuucuucggaaaguaacccucgaaacaaauucauuu

SEQ ID NO: 137 - RNA, 138 nt, Artificial Sequence
  engineered tracrRNA(mature form, 2nt deletion in the first region)
ucacugauaaaguggagaaccgcuucaccaaaagcugucccuuaggggauuagaacuugagugaaggugggcugcuugcaucagccuaaugucgagaagugcuuucuucggaaaguaacccucgaaacaaauucauuu

SEQ ID NO: 138 - RNA, 139 nt, Artificial Sequence
  engineered tracrRNA(mature form, 1nt deletion in the first region)
uucacugauaaaguggagaaccgcuucaccaaaagcugucccuuaggggauuagaacuugagugaaggugggcugcuugcaucagccuaaugucgagaagugcuuucuucggaaaguaacccucgaaacaaauucauuu

SEQ ID NO: 139 - RNA, 117 nt, Artificial Sequence
  engineered tracrRNA(mature form, 10bp deletion in the second region)
cuucacugauaaaguggagaaccgcuucaccauuagugagugaaggugggcugcuugcaucagccuaaugucgagaagugcuuucuucggaaaguaacccucgaaacaaauucauuu

SEQ ID NO: 140 - RNA, 119 nt, Artificial Sequence
  engineered tracrRNA(mature form, 9bp deletion in the second region)
cuucacugauaaaguggagaaccgcuucaccaauuaguugagugaaggugggcugcuugcaucagccuaaugucgagaagugcuuucuucggaaaguaacccucgaaacaaauucauuu

SEQ ID NO: 141 - RNA, 122 nt, Artificial Sequence
  engineered tracrRNA(mature form, 8bp deletion in the second region)
cuucacugauaaaguggagaaccgcuucaccaaauuagacuugagugaaggugggcugcuugcaucagccuaaugucgagaagugcuuucuucggaaaguaacccucgaaacaaauucauuu

SEQ ID NO: 142 - RNA, 125 nt, Artificial Sequence
  engineered tracrRNA(mature form, 7bp deletion in the second region)
cuucacugauaaaguggagaaccgcuucaccaaaaguuagaacuugagugaaggugggcugcuugcaucagccuaaugucgagaagugcuuucuucggaaaguaacccucgaaacaaauucauuu

SEQ ID NO: 143 - RNA, 127 nt, Artificial Sequence
  engineered tracrRNA(mature form, 6bp deletion in the second region)
cuucacugauaaaguggagaaccgcuucaccaaaagcuuaggaacuugagugaaggugggcugcuugcaucagccuaaugucgagaagugcuuucuucggaaaguaacccucgaaacaaauucauuu

SEQ ID NO: 144 - RNA, 129 nt, Artificial Sequence
  engineered tracrRNA(mature form, 5bp deletion in the second region)
cuucacugauaaaguggagaaccgcuucaccaaaagcuuuagagaacuugagugaaggugggcugcuugcaucagccuaaugucgagaagugcuuucuucggaaaguaacccucgaaacaaauucauuu

SEQ ID NO: 145 - RNA, 132 nt, Artificial Sequence
  engineered tracrRNA(mature form, 4bp deletion in the second region)
cuucacugauaaaguggagaaccgcuucaccaaaagcuguuaguuagaacuugagugaaggugggcugcuugcaucagccuaaugucgagaagugcuuucuucggaaaguaacccucgaaacaaauucauuu

SEQ ID NO: 146 - RNA, 131 nt, Artificial Sequence
  engineered tracrRNA(mature form, 4bp+1nt deletion in the second region)
cuucacugauaaaguggagaaccgcuucaccaaaagcuguuaguagaacuugagugaaggugggcugcuugcaucagccuaaugucgagaagugcuuucuucggaaaguaacccucgaaacaaauucauuu

SEQ ID NO: 147 - RNA, 134 nt, Artificial Sequence
  engineered tracrRNA(mature form, 3bp deletion in the second region)
cuucacugauaaaguggagaaccgcuucaccaaaagcuguuuagauuagaacuugagugaaggugggcugcuugcaucagccuaaugucgagaagugcuuucuucggaaaguaacccucgaaacaaauucauuu

SEQ ID NO: 148 - RNA, 136 nt, Artificial Sequence
  engineered tracrRNA(mature form, 2bp deletion in the second region)
cuucacugauaaaguggagaaccgcuucaccaaaagcugucuuaggauuagaacuugagugaaggugggcugcuugcaucagccuaaugucgagaagugcuuucuucggaaaguaacccucgaaacaaauucauuu

SEQ ID NO: 149 - RNA, 138 nt, Artificial Sequence
  engineered tracrRNA(mature form, 1bp deletion in the second region)
cuucacugauaaaguggagaaccgcuucaccaaaagcuguccuuagggauuagaacuugagugaaggugggcugcuugcaucagccuaaugucgagaagugcuuucuucggaaaguaacccucgaaacaaauucauuu

SEQ ID NO: 150 - RNA, 133 nt, Artificial Sequence
  engineered tracrRNA(mature form, 7nt deletion in the fourth region)
cuucacugauaaaguggagaaccgcuucaccaaaagcugucccuuaggggauuagaacuugagugaaggugggcugcuugcaucagccuaaugucgagaagugcuuucuucggaaaguaacccucgaaacaaa

SEQ ID NO: 151 - RNA, 134 nt, Artificial Sequence
  engineered tracrRNA(mature form, 6nt deletion in the fourth region)
cuucacugauaaaguggagaaccgcuucaccaaaagcugucccuuaggggauuagaacuugagugaaggugggcugcuugcaucagccuaaugucgagaagugcuuucuucggaaaguaacccucgaaacaaau

SEQ ID NO: 152 - RNA, 135 nt, Artificial Sequence
  engineered tracrRNA(mature form, 5nt deletion in the fourth region)
cuucacugauaaaguggagaaccgcuucaccaaaagcugucccuuaggggauuagaacuugagugaaggugggcugcuugcaucagccuaaugucgagaagugcuuucuucggaaaguaacccucgaaacaaauu

SEQ ID NO: 153 - RNA, 136 nt, Artificial Sequence
  engineered tracrRNA(mature form, 4nt deletion in the fourth region)
cuucacugauaaaguggagaaccgcuucaccaaaagcugucccuuaggggauuagaacuugagugaaggugggcugcuugcaucagccuaaugucgagaagugcuuucuucggaaaguaacccucgaaacaaauuc

SEQ ID NO: 154 - RNA, 137 nt, Artificial Sequence
  engineered tracrRNA(mature form, 3nt deletion in the fourth region)
cuucacugauaaaguggagaaccgcuucaccaaaagcugucccuuaggggauuagaacuugagugaaggugggcugcuugcaucagccuaaugucgagaagugcuuucuucggaaaguaacccucgaaacaaauuca

SEQ ID NO: 155 - RNA, 138 nt, Artificial Sequence
  engineered tracrRNA(mature form, 2nt deletion in the fourth region)
cuucacugauaaaguggagaaccgcuucaccaaaagcugucccuuaggggauuagaacuugagugaaggugggcugcuugcaucagccuaaugucgagaagugcuuucuucggaaaguaacccucgaaacaaauucau

SEQ ID NO: 156 - RNA, 139 nt, Artificial Sequence
  engineered tracrRNA(mature form, 1nt deletion in the fourth region)
cuucacugauaaaguggagaaccgcuucaccaaaagcugucccuuaggggauuagaacuugagugaaggugggcugcuugcaucagccuaaugucgagaagugcuuucuucggaaaguaacccucgaaacaaauucauu

SEQ ID NO: 157 - RNA, 97 nt, Artificial Sequence
  engineered tracrRNA(mature form, modified first region and modified second region)
accgcuucaccauuagugagugaaggugggcugcuugcaucagccuaaugucgagaagugcuuucuucggaaaguaacccucgaaacaaauucauuu

SEQ ID NO: 158 - RNA, 113 nt, Artificial Sequence
  engineered tracrRNA(mature form, modified first region and modified fourth and fifth region)
accgcuucaccaaaagcugucccuuaggggauuagaacuugagugaaggugggcugcuugcaucagccuaaugucgagaagugcuuucuucggaaaguaacccucgaaacaaa

SEQ ID NO: 159 - RNA, 110 nt, Artificial Sequence
  engineered tracrRNA(mature form, modified second region and modified fourth and fifth region)
cuucacugauaaaguggagaaccgcuucaccauuagugagugaaggugggcugcuugcaucagccuaaugucgagaagugcuuucuucggaaaguaacccucgaaacaaa

SEQ ID NO: 160 - RNA, 90 nt, Artificial Sequence
  engineered tracrRNA(mature form, modified first region, modified second region, modified fourth and fifth region)
accgcuucaccauuagugagugaaggugggcugcuugcaucagccuaaugucgagaagugcuuucuucggaaaguaacccucgaaacaaa

SEQ ID NO: 161 - RNA, 10 nt, Artificial Sequence
  engineered crRNA repeat(mature form, 7nt deletion in the fifth region)
ggaaugcaac

SEQ ID NO: 162 - RNA, 11 nt, Artificial Sequence
  engineered crRNA repeat(mature form, 6nt deletion in the fifth region)
aggaaugcaac

SEQ ID NO: 163 - RNA, 12 nt, Artificial Sequence
  engineered crRNA repeat(mature form, 5nt deletion in the fifth region)
aaggaaugcaac

SEQ ID NO: 164 - RNA, 13 nt, Artificial Sequence
  engineered crRNA repeat(mature form, 4nt deletion in the fifth region)
gaaggaaugcaac

SEQ ID NO: 165 - RNA, 14 nt, Artificial Sequence
  engineered crRNA repeat(mature form, 3nt deletion in the fifth region)
ugaaggaaugcaac

SEQ ID NO: 166 - RNA, 15 nt, Artificial Sequence
  engineered crRNA repeat(mature form, 2nt deletion in the fifth region)
augaaggaaugcaac

SEQ ID NO: 167 - RNA, 16 nt, Artificial Sequence
  engineered crRNA repeat(mature form, 1nt deletion in the fifth region)
aaugaaggaaugcaac

SEQ ID NO: 168 - RNA, 141 nt, Artificial Sequence
  engineered scaffold(mature form, 20nt deletion in the first region)
accgcuucaccaaaagcugucccuuaggggauuagaacuugagugaaggugggcugcuugcaucagccuaaugucgagaagugcuuucuucggaaaguaacccucgaaacaaauucauuugaaagaaugaaggaaugcaac

SEQ ID NO: 169 - RNA, 142 nt, Artificial Sequence
  engineered scaffold(mature form, 19nt deletion in the first region)
aaccgcuucaccaaaagcugucccuuaggggauuagaacuugagugaaggugggcugcuugcaucagccuaaugucgagaagugcuuucuucggaaaguaacccucgaaacaaauucauuugaaagaaugaaggaaugcaac

SEQ ID NO: 170 - RNA, 143 nt, Artificial Sequence
  engineered scaffold(mature form, 18nt deletion in the first region)
gaaccgcuucaccaaaagcugucccuuaggggauuagaacuugagugaaggugggcugcuugcaucagccuaaugucgagaagugcuuucuucggaaaguaacccucgaaacaaauucauuugaaagaaugaaggaaugcaac

SEQ ID NO: 171 - RNA, 144 nt, Artificial Sequence
  engineered scaffold(mature form, 17nt deletion in the first region)
agaaccgcuucaccaaaagcugucccuuaggggauuagaacuugagugaaggugggcugcuugcaucagccuaaugucgagaagugcuuucuucggaaaguaacccucgaaacaaauucauuugaaagaaugaaggaaugcaac

SEQ ID NO: 172 - RNA, 145 nt, Artificial Sequence
  engineered scaffold(mature form, 16nt deletion in the first region)
gagaaccgcuucaccaaaagcugucccuuaggggauuagaacuugagugaaggugggcugcuugcaucagccuaaugucgagaagugcuuucuucggaaaguaacccucgaaacaaauucauuugaaagaaugaaggaaugcaac

SEQ ID NO: 173 - RNA, 146 nt, Artificial Sequence
  engineered scaffold(mature form, 15nt deletion in the first region)
ggagaaccgcuucaccaaaagcugucccuuaggggauuagaacuugagugaaggugggcugcuugcaucagccuaaugucgagaagugcuuucuucggaaaguaacccucgaaacaaauucauuugaaagaaugaaggaaugcaac

SEQ ID NO: 174 - RNA, 147 nt, Artificial Sequence
  engineered scaffold(mature form, 14nt deletion in the first region)
uggagaaccgcuucaccaaaagcugucccuuaggggauuagaacuugagugaaggugggcugcuugcaucagccuaaugucgagaagugcuuucuucggaaaguaacccucgaaacaaauucauuugaaagaaugaaggaaugcaac

SEQ ID NO: 175 - RNA, 148 nt, Artificial Sequence
  engineered scaffold(mature form, 13nt deletion in the first region)
guggagaaccgcuucaccaaaagcugucccuuaggggauuagaacuugagugaaggugggcugcuugcaucagccuaaugucgagaagugcuuucuucggaaaguaacccucgaaacaaauucauuugaaagaaugaaggaaugcaac

SEQ ID NO: 176 - RNA, 149 nt, Artificial Sequence
  engineered scaffold(mature form, 12nt deletion in the first region)
aguggagaaccgcuucaccaaaagcugucccuuaggggauuagaacuugagugaaggugggcugcuugcaucagccuaaugucgagaagugcuuucuucggaaaguaacccucgaaacaaauucauuugaaagaaugaaggaaugcaac

SEQ ID NO: 177 - RNA, 150 nt, Artificial Sequence
  engineered scaffold(mature form, 11nt deletion in the first region)
aaguggagaaccgcuucaccaaaagcugucccuuaggggauuagaacuugagugaaggugggcugcuugcaucagccuaaugucgagaagugcuuucuucggaaaguaacccucgaaacaaauucauuugaaagaaugaaggaaugcaac

SEQ ID NO: 178 - RNA, 151 nt, Artificial Sequence
  engineered scaffold(mature form, 10nt deletion in the first region)
aaaguggagaaccgcuucaccaaaagcugucccuuaggggauuagaacuugagugaaggugggcugcuugcaucagccuaaugucgagaagugcuuucuucggaaaguaacccucgaaacaaauucauuugaaagaaugaaggaaugcaac

SEQ ID NO: 179 - RNA, 152 nt, Artificial Sequence
  engineered scaffold(mature form, 9nt deletion in the first region)
uaaaguggagaaccgcuucaccaaaagcugucccuuaggggauuagaacuugagugaaggugggcugcuugcaucagccuaaugucgagaagugcuuucuucggaaaguaacccucgaaacaaauucauuugaaagaaugaaggaaugcaac

SEQ ID NO: 180 - RNA, 153 nt, Artificial Sequence
  engineered scaffold(mature form, 8nt deletion in the first region)
auaaaguggagaaccgcuucaccaaaagcugucccuuaggggauuagaacuugagugaaggugggcugcuugcaucagccuaaugucgagaagugcuuucuucggaaaguaacccucgaaacaaauucauuugaaagaaugaaggaaugcaac

SEQ ID NO: 181 - RNA, 154 nt, Artificial Sequence
  engineered scaffold(mature form, 7nt deletion in the first region)
gauaaaguggagaaccgcuucaccaaaagcugucccuuaggggauuagaacuugagugaaggugggcugcuugcaucagccuaaugucgagaagugcuuucuucggaaaguaacccucgaaacaaauucauuugaaagaaugaaggaaugcaac

SEQ ID NO: 182 - RNA, 155 nt, Artificial Sequence
  engineered scaffold(mature form, 6nt deletion in the first region)
ugauaaaguggagaaccgcuucaccaaaagcugucccuuaggggauuagaacuugagugaaggugggcugcuugcaucagccuaaugucgagaagugcuuucuucggaaaguaacccucgaaacaaauucauuugaaagaaugaaggaaugcaac

SEQ ID NO: 183 - RNA, 156 nt, Artificial Sequence
  engineered scaffold(mature form, 5nt deletion in the first region)
cugauaaaguggagaaccgcuucaccaaaagcugucccuuaggggauuagaacuugagugaaggugggcugcuugcaucagccuaaugucgagaagugcuuucuucggaaaguaacccucgaaacaaauucauuugaaagaaugaaggaaugcaac

SEQ ID NO: 184 - RNA, 157 nt, Artificial Sequence
  engineered scaffold(mature form, 4nt deletion in the first region)
acugauaaaguggagaaccgcuucaccaaaagcugucccuuaggggauuagaacuugagugaaggugggcugcuugcaucagccuaaugucgagaagugcuuucuucggaaaguaacccucgaaacaaauucauuugaaagaaugaaggaaugcaac

SEQ ID NO: 185 - RNA, 158 nt, Artificial Sequence
  engineered scaffold(mature form, 3nt deletion in the first region)
cacugauaaaguggagaaccgcuucaccaaaagcugucccuuaggggauuagaacuugagugaaggugggcugcuugcaucagccuaaugucgagaagugcuuucuucggaaaguaacccucgaaacaaauucauuugaaagaaugaaggaaugcaac

SEQ ID NO: 186 - RNA, 159 nt, Artificial Sequence
  engineered scaffold(mature form, 2nt deletion in the first region)
ucacugauaaaguggagaaccgcuucaccaaaagcugucccuuaggggauuagaacuugagugaaggugggcugcuugcaucagccuaaugucgagaagugcuuucuucggaaaguaacccucgaaacaaauucauuugaaagaaugaaggaaugcaac

SEQ ID NO: 187 - RNA, 160 nt, Artificial Sequence
  engineered scaffold(mature form, 1nt deletion in the first region)
uucacugauaaaguggagaaccgcuucaccaaaagcugucccuuaggggauuagaacuugagugaaggugggcugcuugcaucagccuaaugucgagaagugcuuucuucggaaaguaacccucgaaacaaauucauuugaaagaaugaaggaaugcaac

SEQ ID NO: 188 - RNA, 138 nt, Artificial Sequence
  engineered scaffold(mature form, 11bp deletion in the second region)
cuucacugauaaaguggagaaccgcuucaccauuagugagugaaggugggcugcuugcaucagccuaaugucgagaagugcuuucuucggaaaguaacccucgaaacaaauucauuugaaagaaugaaggaaugcaac

SEQ ID NO: 189 - RNA, 140 nt, Artificial Sequence
  engineered scaffold(mature form, 10bp deletion in the second region)
cuucacugauaaaguggagaaccgcuucaccaauuaguugagugaaggugggcugcuugcaucagccuaaugucgagaagugcuuucuucggaaaguaacccucgaaacaaauucauuugaaagaaugaaggaaugcaac

SEQ ID NO: 190 - RNA, 142 nt, Artificial Sequence
  engineered scaffold(mature form, 9bp deletion in the second region)
cuucacugauaaaguggagaaccgcuucaccaaauuagcuugagugaaggugggcugcuugcaucagccuaaugucgagaagugcuuucuucggaaaguaacccucgaaacaaauucauuugaaagaaugaaggaaugcaac

SEQ ID NO: 191 - RNA, 144 nt, Artificial Sequence
  engineered scaffold(mature form, 8bp deletion in the second region)
cuucacugauaaaguggagaaccgcuucaccaaaauuagacuugagugaaggugggcugcuugcaucagccuaaugucgagaagugcuuucuucggaaaguaacccucgaaacaaauucauuugaaagaaugaaggaaugcaac

SEQ ID NO: 192 - RNA, 146 nt, Artificial Sequence
  engineered scaffold(mature form, 7bp deletion in the second region)
cuucacugauaaaguggagaaccgcuucaccaaaaguuagaacuugagugaaggugggcugcuugcaucagccuaaugucgagaagugcuuucuucggaaaguaacccucgaaacaaauucauuugaaagaaugaaggaaugcaac

SEQ ID NO: 193 - RNA, 148 nt, Artificial Sequence
  engineered scaffold(mature form, 6bp deletion in the second region)
cuucacugauaaaguggagaaccgcuucaccaaaagcuuaggaacuugagugaaggugggcugcuugcaucagccuaaugucgagaagugcuuucuucggaaaguaacccucgaaacaaauucauuugaaagaaugaaggaaugcaac

SEQ ID NO: 194 - RNA, 150 nt, Artificial Sequence
  engineered scaffold(mature form, 5bp deletion in the second region)
cuucacugauaaaguggagaaccgcuucaccaaaagcuuuagagaacuugagugaaggugggcugcuugcaucagccuaaugucgagaagugcuuucuucggaaaguaacccucgaaacaaauucauuugaaagaaugaaggaaugcaac

SEQ ID NO: 195 - RNA, 152 nt, Artificial Sequence
  engineered scaffold(mature form, 4bp deletion in the second region)
cuucacugauaaaguggagaaccgcuucaccaaaagcuguuaguagaacuugagugaaggugggcugcuugcaucagccuaaugucgagaagugcuuucuucggaaaguaacccucgaaacaaauucauuugaaagaaugaaggaaugcaac

SEQ ID NO: 196 - RNA, 153 nt, Artificial Sequence
  engineered scaffold(mature form, 4bp+1nt deletion in the second region)
cuucacugauaaaguggagaaccgcuucaccaaaagcuguuaguuagaacuugagugaaggugggcugcuugcaucagccuaaugucgagaagugcuuucuucggaaaguaacccucgaaacaaauucauuugaaagaaugaaggaaugcaac

SEQ ID NO: 197 - RNA, 155 nt, Artificial Sequence
  engineered scaffold(mature form, 3bp deletion in the second region)
cuucacugauaaaguggagaaccgcuucaccaaaagcuguuuagauuagaacuugagugaaggugggcugcuugcaucagccuaaugucgagaagugcuuucuucggaaaguaacccucgaaacaaauucauuugaaagaaugaaggaaugcaac

SEQ ID NO: 198 - RNA, 157 nt, Artificial Sequence
  engineered scaffold(mature form, 2bp deletion in the second region)
cuucacugauaaaguggagaaccgcuucaccaaaagcugucuuaggauuagaacuugagugaaggugggcugcuugcaucagccuaaugucgagaagugcuuucuucggaaaguaacccucgaaacaaauucauuugaaagaaugaaggaaugcaac

SEQ ID NO: 199 - RNA, 159 nt, Artificial Sequence
  engineered scaffold(mature form, 1bp deletion in the second region)
cuucacugauaaaguggagaaccgcuucaccaaaagcuguccuuagggauuagaacuugagugaaggugggcugcuugcaucagccuaaugucgagaagugcuuucuucggaaaguaacccucgaaacaaauucauuugaaagaaugaaggaaugcaac

SEQ ID NO: 200 - RNA, 147 nt, Artificial Sequence
  engineered scaffold(mature form, 7bp deletion in the fourth and fifth region)
cuucacugauaaaguggagaaccgcuucaccaaaagcugucccuuaggggauuagaacuugagugaaggugggcugcuugcaucagccuaaugucgagaagugcuuucuucggaaaguaacccucgaaacaaagaaaggaaugcaac

SEQ ID NO: 201 - RNA, 149 nt, Artificial Sequence
  engineered scaffold(mature form, 6bp deletion in the fourth and fifth region)
cuucacugauaaaguggagaaccgcuucaccaaaagcugucccuuaggggauuagaacuugagugaaggugggcugcuugcaucagccuaaugucgagaagugcuuucuucggaaaguaacccucgaaacaaaugaaaaggaaugcaac

SEQ ID NO: 202 - RNA, 151 nt, Artificial Sequence
  engineered scaffold(mature form, 5bp deletion in the fourth and fifth region)
cuucacugauaaaguggagaaccgcuucaccaaaagcugucccuuaggggauuagaacuugagugaaggugggcugcuugcaucagccuaaugucgagaagugcuuucuucggaaaguaacccucgaaacaaauugaaaaaggaaugcaac

SEQ ID NO: 203 - RNA, 153 nt, Artificial Sequence
  engineered scaffold(mature form, 4bp deletion in the fourth and fifth region)
cuucacugauaaaguggagaaccgcuucaccaaaagcugucccuuaggggauuagaacuugagugaaggugggcugcuugcaucagccuaaugucgagaagugcuuucuucggaaaguaacccucgaaacaaauucgaaagaaggaaugcaac

SEQ ID NO: 204 - RNA, 155 nt, Artificial Sequence
  engineered scaffold(mature form, 3bp deletion in the fourth and fifth region)
cuucacugauaaaguggagaaccgcuucaccaaaagcugucccuuaggggauuagaacuugagugaaggugggcugcuugcaucagccuaaugucgagaagugcuuucuucggaaaguaacccucgaaacaaauucagaaaugaaggaaugcaac

SEQ ID NO: 205 - RNA, 157 nt, Artificial Sequence
  engineered scaffold(mature form, 2bp deletion in the fourth and fifth region)
cuucacugauaaaguggagaaccgcuucaccaaaagcugucccuuaggggauuagaacuugagugaaggugggcugcuugcaucagccuaaugucgagaagugcuuucuucggaaaguaacccucgaaacaaauucaugaaaaugaaggaaugcaac

SEQ ID NO: 206 - RNA, 159 nt, Artificial Sequence
  engineered scaffold(mature form, 1bp deletion in the fourth and fifth region)
cuucacugauaaaguggagaaccgcuucaccaaaagcugucccuuaggggauuagaacuugagugaaggugggcugcuugcaucagccuaaugucgagaagugcuuucuucggaaaguaacccucgaaacaaauucauugaaaaaugaaggaaugcaac

SEQ ID NO: 207 - RNA, 118 nt, Artificial Sequence
  engineered scaffold(mature form, modified first and second region)
accgcuucaccauuagugagugaaggugggcugcuugcaucagccuaaugucgagaagugcuuucuucggaaaguaacccucgaaacaaauucauuugaaagaaugaaggaaugcaac

SEQ ID NO: 208 - RNA, 127 nt, Artificial Sequence
  engineered scaffold(mature form, modified first, fourth and fifth region)
accgcuucaccaaaagcugucccuuaggggauuagaacuugagugaaggugggcugcuugcaucagccuaaugucgagaagugcuuucuucggaaaguaacccucgaaacaaagaaaggaaugcaac

SEQ ID NO: 209 - RNA, 121 nt, Artificial Sequence
  engineered scaffold(mature form, modified second, fourth and fifth region)
cuucacugauaaaguggagaaccgcuucacuuagagugaagguggggcugcuugcaucagccuaaugucgagaagugcuuucuucggaaaguaacccucgaaacaaagaaaggaaugcaac

SEQ ID NO: 210 - RNA, 101 nt, Artificial Sequence
  engineered scaffold(mature form, modified first, second, fourth and fifth region)
accgcuucacuuagagugaagguggggcugcuugcaucagccuaaugucgagaagugcuuucuucggaaaguaacccucgaaacaaagaaaggaaugcaac

SEQ ID NO: 211 - RNA, 189 nt, Artificial Sequence
  sgRNA(mature form, 1nt deletion in the first region)
uucacugauaaaguggagaaccgcuucaccaaaagcugucccuuaggggauuagaacuugagugaaggugggcugcuugcaucagccuaaugucgagaagugcuuucuucggaaaguaacccucgaaacaaauucauuugaaagaaugaaggaaugcaacnnnnnnnnnnnnnnnnnnnnuuuuauuuu

SEQ ID NO: 212 - RNA, 188 nt, Artificial Sequence
  sgRNA(mature form, 2nt deletion in the first region)
ucacugauaaaguggagaaccgcuucaccaaaagcugucccuuaggggauuagaacuugagugaaggugggcugcuugcaucagccuaaugucgagaagugcuuucuucggaaaguaacccucgaaacaaauucauuugaaagaaugaaggaaugcaacnnnnnnnnnnnnnnnnnnnnuuuuauuuu

SEQ ID NO: 213 - RNA, 187 nt, Artificial Sequence
  sgRNA(mature form, 3nt deletion in the first region)
cacugauaaaguggagaaccgcuucaccaaaagcugucccuuaggggauuagaacuugagugaaggugggcugcuugcaucagccuaaugucgagaagugcuuucuucggaaaguaacccucgaaacaaauucauuugaaagaaugaaggaaugcaacnnnnnnnnnnnnnnnnnnnnuuuuauuuu

SEQ ID NO: 214 - RNA, 186 nt, Artificial Sequence
  sgRNA(mature form, 4nt deletion in the first region)
acugauaaaguggagaaccgcuucaccaaaagcugucccuuaggggauuagaacuugagugaaggugggcugcuugcaucagccuaaugucgagaagugcuuucuucggaaaguaacccucgaaacaaauucauuugaaagaaugaaggaaugcaacnnnnnnnnnnnnnnnnnnnnuuuuauuuu

SEQ ID NO: 215 - RNA, 185 nt, Artificial Sequence
  sgRNA(mature form, 5nt deletion in the first region)
cugauaaaguggagaaccgcuucaccaaaagcugucccuuaggggauuagaacuugagugaaggugggcugcuugcaucagccuaaugucgagaagugcuuucuucggaaaguaacccucgaaacaaauucauuugaaagaaugaaggaaugcaacnnnnnnnnnnnnnnnnnnnnuuuuauuuu

SEQ ID NO: 216 - RNA, 184 nt, Artificial Sequence
  sgRNA(mature form, 6nt deletion in the first region)
ugauaaaguggagaaccgcuucaccaaaagcugucccuuaggggauuagaacuugagugaaggugggcugcuugcaucagccuaaugucgagaagugcuuucuucggaaaguaacccucgaaacaaauucauuugaaagaaugaaggaaugcaacnnnnnnnnnnnnnnnnnnnnuuuuauuuu

SEQ ID NO: 217 - RNA, 183 nt, Artificial Sequence
  sgRNA(mature form, 7nt deletion in the first region)
gauaaaguggagaaccgcuucaccaaaagcugucccuuaggggauuagaacuugagugaaggugggcugcuugcaucagccuaaugucgagaagugcuuucuucggaaaguaacccucgaaacaaauucauuugaaagaaugaaggaaugcaacnnnnnnnnnnnnnnnnnnnnuuuuauuuu

SEQ ID NO: 218 - RNA, 182 nt, Artificial Sequence
  sgRNA(mature form, 8nt deletion in the first region)
auaaaguggagaaccgcuucaccaaaagcugucccuuaggggauuagaacuugagugaaggugggcugcuugcaucagccuaaugucgagaagugcuuucuucggaaaguaacccucgaaacaaauucauuugaaagaaugaaggaaugcaacnnnnnnnnnnnnnnnnnnnnuuuuauuuu

SEQ ID NO: 219 - RNA, 181 nt, Artificial Sequence
  sgRNA(mature form, 9nt deletion in the first region)
uaaaguggagaaccgcuucaccaaaagcugucccuuaggggauuagaacuugagugaaggugggcugcuugcaucagccuaaugucgagaagugcuuucuucggaaaguaacccucgaaacaaauucauuugaaagaaugaaggaaugcaacnnnnnnnnnnnnnnnnnnnnuuuuauuuu

SEQ ID NO: 220 - RNA, 180 nt, Artificial Sequence
  sgRNA(mature form, 10nt deletion in the first region)
aaaguggagaaccgcuucaccaaaagcugucccuuaggggauuagaacuugagugaaggugggcugcuugcaucagccuaaugucgagaagugcuuucuucggaaaguaacccucgaaacaaauucauuugaaagaaugaaggaaugcaacnnnnnnnnnnnnnnnnnnnnuuuuauuuu

SEQ ID NO: 221 - RNA, 179 nt, Artificial Sequence
  sgRNA(mature form, 11nt deletion in the first region)
aaguggagaaccgcuucaccaaaagcugucccuuaggggauuagaacuugagugaaggugggcugcuugcaucagccuaaugucgagaagugcuuucuucggaaaguaacccucgaaacaaauucauuugaaagaaugaaggaaugcaacnnnnnnnnnnnnnnnnnnnnuuuuauuuu

SEQ ID NO: 222 - RNA, 178 nt, Artificial Sequence
  sgRNA(mature form, 12nt deletion in the first region)
aguggagaaccgcuucaccaaaagcugucccuuaggggauuagaacuugagugaaggugggcugcuugcaucagccuaaugucgagaagugcuuucuucggaaaguaacccucgaaacaaauucauuugaaagaaugaaggaaugcaacnnnnnnnnnnnnnnnnnnnnuuuuauuuu

SEQ ID NO: 223 - RNA, 177 nt, Artificial Sequence
  sgRNA(mature form, 13nt deletion in the first region)
guggagaaccgcuucaccaaaagcugucccuuaggggauuagaacuugagugaaggugggcugcuugcaucagccuaaugucgagaagugcuuucuucggaaaguaacccucgaaacaaauucauuugaaagaaugaaggaaugcaacnnnnnnnnnnnnnnnnnnnnuuuuauuuu

SEQ ID NO: 224 - RNA, 176 nt, Artificial Sequence
  sgRNA(mature form, 14nt deletion in the first region)
uggagaaccgcuucaccaaaagcugucccuuaggggauuagaacuugagugaaggugggcugcuugcaucagccuaaugucgagaagugcuuucuucggaaaguaacccucgaaacaaauucauuugaaagaaugaaggaaugcaacnnnnnnnnnnnnnnnnnnnnuuuuauuuu

SEQ ID NO: 225 - RNA, 175 nt, Artificial Sequence
  sgRNA(mature form, 15nt deletion in the first region)
ggagaaccgcuucaccaaaagcugucccuuaggggauuagaacuugagugaaggugggcugcuugcaucagccuaaugucgagaagugcuuucuucggaaaguaacccucgaaacaaauucauuugaaagaaugaaggaaugcaacnnnnnnnnnnnnnnnnnnnnuuuuauuuu

SEQ ID NO: 226 - RNA, 174 nt, Artificial Sequence
  sgRNA(mature form, 16nt deletion in the first region)
gagaaccgcuucaccaaaagcugucccuuaggggauuagaacuugagugaaggugggcugcuugcaucagccuaaugucgagaagugcuuucuucggaaaguaacccucgaaacaaauucauuugaaagaaugaaggaaugcaacnnnnnnnnnnnnnnnnnnnnuuuuauuuu

SEQ ID NO: 227 - RNA, 173 nt, Artificial Sequence
  sgRNA(mature form, 17nt deletion in the first region)
agaaccgcuucaccaaaagcugucccuuaggggauuagaacuugagugaaggugggcugcuugcaucagccuaaugucgagaagugcuuucuucggaaaguaacccucgaaacaaauucauuugaaagaaugaaggaaugcaacnnnnnnnnnnnnnnnnnnnnuuuuauuuu

SEQ ID NO: 228 - RNA, 172 nt, Artificial Sequence
  sgRNA(mature form, 18nt deletion in the first region)
gaaccgcuucaccaaaagcugucccuuaggggauuagaacuugagugaaggugggcugcuugcaucagccuaaugucgagaagugcuuucuucggaaaguaacccucgaaacaaauucauuugaaagaaugaaggaaugcaacnnnnnnnnnnnnnnnnnnnnuuuuauuuu

SEQ ID NO: 229 - RNA, 171 nt, Artificial Sequence
  sgRNA(mature form, 19nt deletion in the first region)
aaccgcuucaccaaaagcugucccuuaggggauuagaacuugagugaaggugggcugcuugcaucagccuaaugucgagaagugcuuucuucggaaaguaacccucgaaacaaauucauuugaaagaaugaaggaaugcaacnnnnnnnnnnnnnnnnnnnnuuuuauuuu

SEQ ID NO: 230 - RNA, 170 nt, Artificial Sequence
  sgRNA(mature form, 20nt deletion in the first region)
accgcuucaccaaaagcugucccuuaggggauuagaacuugagugaaggugggcugcuugcaucagccuaaugucgagaagugcuuucuucggaaaguaacccucgaaacaaauucauuugaaagaaugaaggaaugcaacnnnnnnnnnnnnnnnnnnnnuuuuauuuu

SEQ ID NO: 231 - RNA, 188 nt, Artificial Sequence
  sgRNA(mature form, 1bp deletion in the second region)
cuucacugauaaaguggagaaccgcuucaccaaaagcuguccuuagggauuagaacuugagugaaggugggcugcuugcaucagccuaaugucgagaagugcuuucuucggaaaguaacccucgaaacaaauucauuugaaagaaugaaggaaugcaacnnnnnnnnnnnnnnnnnnnnuuuuauuuu

SEQ ID NO: 232 - RNA, 186 nt, Artificial Sequence
  sgRNA(mature form, 2bp deletion in the second region)
cuucacugauaaaguggagaaccgcuucaccaaaagcugucuuaggauuagaacuugagugaaggugggcugcuugcaucagccuaaugucgagaagugcuuucuucggaaaguaacccucgaaacaaauucauuugaaagaaugaaggaaugcaacnnnnnnnnnnnnnnnnnnnnuuuuauuuu

SEQ ID NO: 233 - RNA, 184 nt, Artificial Sequence
  sgRNA(mature form, 3bp deletion in the second region)
cuucacugauaaaguggagaaccgcuucaccaaaagcuguuuagauuagaacuugagugaaggugggcugcuugcaucagccuaaugucgagaagugcuuucuucggaaaguaacccucgaaacaaauucauuugaaagaaugaaggaaugcaacnnnnnnnnnnnnnnnnnnnnuuuuauuuu

SEQ ID NO: 234 - RNA, 182 nt, Artificial Sequence
  sgRNA(mature form, 4bp+1nt deletion in the second region)
cuucacugauaaaguggagaaccgcuucaccaaaagcuguuaguuagaacuugagugaaggugggcugcuugcaucagccuaaugucgagaagugcuuucuucggaaaguaacccucgaaacaaauucauuugaaagaaugaaggaaugcaacnnnnnnnnnnnnnnnnnnnnuuuuauuuu

SEQ ID NO: 235 - RNA, 181 nt, Artificial Sequence
  sgRNA(mature form, 4bp deletion in the second region)
cuucacugauaaaguggagaaccgcuucaccaaaagcuguuaguagaacuugagugaaggugggcugcuugcaucagccuaaugucgagaagugcuuucuucggaaaguaacccucgaaacaaauucauuugaaagaaugaaggaaugcaacnnnnnnnnnnnnnnnnnnnnuuuuauuuu

SEQ ID NO: 236 - RNA, 179 nt, Artificial Sequence
  sgRNA(mature form, 5bp deletion in the second region)
cuucacugauaaaguggagaaccgcuucaccaaaagcuuuagagaacuugagugaaggugggcugcuugcaucagccuaaugucgagaagugcuuucuucggaaaguaacccucgaaacaaauucauuugaaagaaugaaggaaugcaacnnnnnnnnnnnnnnnnnnnnuuuuauuuu

SEQ ID NO: 237 - RNA, 177 nt, Artificial Sequence
  sgRNA(mature form, 6bp deletion in the second region)
cuucacugauaaaguggagaaccgcuucaccaaaagcuuaggaacuugagugaaggugggcugcuugcaucagccuaaugucgagaagugcuuucuucggaaaguaacccucgaaacaaauucauuugaaagaaugaaggaaugcaacnnnnnnnnnnnnnnnnnnnnuuuuauuuu

SEQ ID NO: 238 - RNA, 175 nt, Artificial Sequence
  sgRNA(mature form, 7bp deletion in the second region)
cuucacugauaaaguggagaaccgcuucaccaaaaguuagaacuugagugaaggugggcugcuugcaucagccuaaugucgagaagugcuuucuucggaaaguaacccucgaaacaaauucauuugaaagaaugaaggaaugcaacnnnnnnnnnnnnnnnnnnnnuuuuauuuu

SEQ ID NO: 239 - RNA, 173 nt, Artificial Sequence
  sgRNA(mature form, 8bp deletion in the second region)
cuucacugauaaaguggagaaccgcuucaccaaaauuagacuugagugaaggugggcugcuugcaucagccuaaugucgagaagugcuuucuucggaaaguaacccucgaaacaaauucauuugaaagaaugaaggaaugcaacnnnnnnnnnnnnnnnnnnnnuuuuauuuu

SEQ ID NO: 240 - RNA, 171 nt, Artificial Sequence
  sgRNA(mature form, 9bp deletion in the second region)
cuucacugauaaaguggagaaccgcuucaccaaauuagcuugagugaaggugggcugcuugcaucagccuaaugucgagaagugcuuucuucggaaaguaacccucgaaacaaauucauuugaaagaaugaaggaaugcaacnnnnnnnnnnnnnnnnnnnnuuuuauuuu

SEQ ID NO: 241 - RNA, 169 nt, Artificial Sequence
  sgRNA(mature form, 10bp deletion in the second region)
cuucacugauaaaguggagaaccgcuucaccaauuaguugagugaaggugggcugcuugcaucagccuaaugucgagaagugcuuucuucggaaaguaacccucgaaacaaauucauuugaaagaaugaaggaaugcaacnnnnnnnnnnnnnnnnnnnnuuuuauuuu

SEQ ID NO: 242 - RNA, 167 nt, Artificial Sequence
  sgRNA(mature form, 11bp deletion in the second region)
cuucacugauaaaguggagaaccgcuucaccauuagugagugaaggugggcugcuugcaucagccuaaugucgagaagugcuuucuucggaaaguaacccucgaaacaaauucauuugaaagaaugaaggaaugcaacnnnnnnnnnnnnnnnnnnnnuuuuauuuu

SEQ ID NO: 243 - RNA, 188 nt, Artificial Sequence
  sgRNA(mature form, 1bp deletion in the fourth and fifth region)
cuucacugauaaaguggagaaccgcuucaccaaaagcugucccuuaggggauuagaacuugagugaaggugggcugcuugcaucagccuaaugucgagaagugcuuucuucggaaaguaacccucgaaacaaauucauugaaaaaugaaggaaugcaacnnnnnnnnnnnnnnnnnnnnuuuuauuuu

SEQ ID NO: 244 - RNA, 186 nt, Artificial Sequence
  sgRNA(mature form, 2bp deletion in the fourth and fifth region)
cuucacugauaaaguggagaaccgcuucaccaaaagcugucccuuaggggauuagaacuugagugaaggugggcugcuugcaucagccuaaugucgagaagugcuuucuucggaaaguaacccucgaaacaaauucaugaaaaugaaggaaugcaacnnnnnnnnnnnnnnnnnnnnuuuuauuuu

SEQ ID NO: 245 - RNA, 184 nt, Artificial Sequence
  sgRNA(mature form, 3bp deletion in the fourth and fifth region)
cuucacugauaaaguggagaaccgcuucaccaaaagcugucccuuaggggauuagaacuugagugaaggugggcugcuugcaucagccuaaugucgagaagugcuuucuucggaaaguaacccucgaaacaaauucagaaaugaaggaaugcaacnnnnnnnnnnnnnnnnnnnnuuuuauuuu

SEQ ID NO: 246 - RNA, 182 nt, Artificial Sequence
  sgRNA(mature form, 4bp deletion in the fourth and fifth region)
cuucacugauaaaguggagaaccgcuucaccaaaagcugucccuuaggggauuagaacuugagugaaggugggcugcuugcaucagccuaaugucgagaagugcuuucuucggaaaguaacccucgaaacaaauucgaaagaaggaaugcaacnnnnnnnnnnnnnnnnnnnnuuuuauuuu

SEQ ID NO: 247 - RNA, 180 nt, Artificial Sequence
  sgRNA(mature form, 5bp deletion in the fourth and fifth region)
cuucacugauaaaguggagaaccgcuucaccaaaagcugucccuuaggggauuagaacuugagugaaggugggcugcuugcaucagccuaaugucgagaagugcuuucuucggaaaguaacccucgaaacaaauugaaaaaggaaugcaacnnnnnnnnnnnnnnnnnnnnuuuuauuuu

SEQ ID NO: 248 - RNA, 178 nt, Artificial Sequence
  sgRNA(mature form, 6bp deletion in the fourth and fifth region)
cuucacugauaaaguggagaaccgcuucaccaaaagcugucccuuaggggauuagaacuugagugaaggugggcugcuugcaucagccuaaugucgagaagugcuuucuucggaaaguaacccucgaaacaaaugaaaaggaaugcaacnnnnnnnnnnnnnnnnnnnnuuuuauuuu

SEQ ID NO: 249 - RNA, 176 nt, Artificial Sequence
  sgRNA(mature form, 7bp deletion in the fourth and fifth region)
cuucacugauaaaguggagaaccgcuucaccaaaagcugucccuuaggggauuagaacuugagugaaggugggcugcuugcaucagccuaaugucgagaagugcuuucuucggaaaguaacccucgaaacaaagaaaggaaugcaacnnnnnnnnnnnnnnnnnnnnuuuuauuuu

SEQ ID NO: 250 - RNA, 147 nt, Artificial Sequence
  sgRNA(mature form, modified first and second region)
accgcuucaccauuagugagugaaggugggcugcuugcaucagccuaaugucgagaagugcuuucuucggaaaguaacccucgaaacaaauucauuugaaagaaugaaggaaugcaacnnnnnnnnnnnnnnnnnnnnuuuuauuuu

SEQ ID NO: 251 - RNA, 156 nt, Artificial Sequence
  sgRNA(mature form, modified first, fourth and fifth region)
accgcuucaccaaaagcugucccuuaggggauuagaacuugagugaaggugggcugcuugcaucagccuaaugucgagaagugcuuucuucggaaaguaacccucgaaacaaagaaaggaaugcaacnnnnnnnnnnnnnnnnnnnnuuuuauuuu

SEQ ID NO: 252 - RNA, 153 nt, Artificial Sequence
  sgRNA(mature form, modified second, fourth and fifth region)
cuucacugauaaaguggagaaccgcuucaccauuagugagugaaggugggcugcuugcaucagccuaaugucgagaagugcuuucuucggaaaguaacccucgaaacaaagaaaggaaugcaacnnnnnnnnnnnnnnnnnnnnuuuuauuuu

SEQ ID NO: 253 - RNA, 130 nt, Artificial Sequence
  sgRNA(mature form, modified first, second, fourth and fifth region)
accgcuucacuuagagugaagguggggcugcuugcaucagccuaaugucgagaagugcuuucuucggaaaguaacccucgaaacaaagaaaggaaugcaacnnnnnnnnnnnnnnnnnnnnuuuuauuuu

SEQ ID NO: 254 - RNA, 11 nt, Artificial Sequence
  U-rich tail sequence
uuuauuuauuu

SEQ ID NO: 255 - RNA, 10 nt, Artificial Sequence
  U-rich tail sequence
uuuuauuuuu

SEQ ID NO: 256 - RNA, 11 nt, Artificial Sequence
  U-rich tail sequence
uuuuauuuuuu

SEQ ID NO: 257 - RNA, 11 nt, Artificial Sequence
  U-rich tail sequence
uuuguuuguuu

SEQ ID NO: 258 - RNA, 10 nt, Artificial Sequence
  U-rich tail sequence
uuuuguuuuu

SEQ ID NO: 259 - RNA, 11 nt, Artificial Sequence
  U-rich tail sequence
uuuuguuuuuu

SEQ ID NO: 260 - protein, 529 aa, Artificial Sequence
  Cas14a1 amino acid sequence
MAKNTITKTLKLRIVRPYNSAEVEKIVADEKNNREKIALEKNKDKVKEACSKHLKVAAYCTTQVERNACLFCKARKLDDKFYQKLRGQFPDAVFWQEISEIFRQLQKQAAEIYNQSLIELYYEIFIKGKGIANASSVEHYLSDVCYTRAAELFKNAAIASGLRSKIKSNFRLKELKNMKSGLPTTKSDNFPIPLVKQKGGQYTGFEISNHNSDFIIKIPFGRWQVKKEIDKYRPWEKFDFEQVQKSPKPISLLLSTQRRKRNKGWSKDEGTEAEIKKVMNGDYQTSYIEVKRGSKIGEKSAWMLNLSIDVPKIDKGVDPSIIGGIDVGVKSPLVCAINNAFSRYSISDNDLFHFNKKMFARRRILLKKNRHKRAGHGAKNKLKPITILTEKSERFRKKLIERWACEIADFFIKNKVGTVQMENLESMKRKEDSYFNIRLRGFWPYAEMQNKIEFKLKQYGIEIRKVAPNNTSKTCSKCGHLNNYFNFEYRKKNKFPHFKCEKCNFKENADYNAALNISNPKLKSTKEEP

SEQ ID NO: 261 - protein, 529 aa, Artificial Sequence
  dCas12f1 R490A protein
MAKNTITKTLKLRIVRPYNSAEVEKIVADEKNNREKIALEKNKDKVKEACSKHLKVAAYCTTQVERNACLFCKARKLDDKFYQKLRGQFPDAVFWQEISEIFRQLQKQAAEIYNQSLIELYYEIFIKGKGIANASSVEHYLSDVCYTRAAELFKNAAIASGLRSKIKSNFRLKELKNMKSGLPTTKSDNFPIPLVKQKGGQYTGFEISNHNSDFIIKIPFGRWQVKKEIDKYRPWEKFDFEQVQKSPKPISLLLSTQRRKRNKGWSKDEGTEAEIKKVMNGDYQTSYIEVKRGSKIGEKSAWMLNLSIDVPKIDKGVDPSIIGGIDVGVKSPLVCAINNAFSRYSISDNDLFHFNKKMFARRRILLKKNRHKRAGHGAKNKLKPITILTEKSERFRKKLIERWACEIADFFIKNKVGTVQMENLESMKRKEDSYFNIRLRGFWPYAEMQNKIEFKLKQYGIEIRKVAPNNTSKTCSKCGHLNNYFNFEYAKKNKFPHFKCEKCNFKENADYNAALNISNPKLKSTKEEP

SEQ ID NO: 262 - protein, 529 aa, Artificial Sequence
  dCas12f1 R490Q protein
MAKNTITKTLKLRIVRPYNSAEVEKIVADEKNNREKIALEKNKDKVKEACSKHLKVAAYCTTQVERNACLFCKARKLDDKFYQKLRGQFPDAVFWQEISEIFRQLQKQAAEIYNQSLIELYYEIFIKGKGIANASSVEHYLSDVCYTRAAELFKNAAIASGLRSKIKSNFRLKELKNMKSGLPTTKSDNFPIPLVKQKGGQYTGFEISNHNSDFIIKIPFGRWQVKKEIDKYRPWEKFDFEQVQKSPKPISLLLSTQRRKRNKGWSKDEGTEAEIKKVMNGDYQTSYIEVKRGSKIGEKSAWMLNLSIDVPKIDKGVDPSIIGGIDVGVKSPLVCAINNAFSRYSISDNDLFHFNKKMFARRRILLKKNRHKRAGHGAKNKLKPITILTEKSERFRKKLIERWACEIADFFIKNKVGTVQMENLESMKRKEDSYFNIRLRGFWPYAEMQNKIEFKLKQYGIEIRKVAPNNTSKTCSKCGHLNNYFNFEYQKKNKFPHFKCEKCNFKENADYNAALNISNPKLKSTKEEP

SEQ ID NO: 263 - protein, 536 aa, Artificial Sequence
  N/C-terminal NLS + Cas14a1 amino acid sequence
MAKNTITKTLKLRIVRPYNSAEVEKIVADEKNNREKIALEKNKDKVKEACSKHLKVAAYCTTQVERNACLFCKARKLDDKFYQKLRGQFPDAVFWQEISEIFRQLQKQAAEIYNQSLIELYYEIFIKGKGIANASSVEHYLSDVCYTRAAELFKNAAIASGLRSKIKSNFRLKELKNMKSGLPTTKSDNFPIPLVKQKGGQYTGFEISNHNSDFIIKIPFGRWQVKKEIDKYRPWEKFDFEQVQKSPKPISLLLSTQRRKRNKGWSKDEGTEAEIKKVMNGDYQTSYIEVKRGSKIGEKSAWMLNLSIDVPKIDKGVDPSIIGGIDVGVKSPLVCAINNAFSRYSISDNDLFHFNKKMFARRRILLKKNRHKRAGHGAKNKLKPITILTEKSERFRKKLIERWACEIADFFIKNKVGTVQMENLESMKRKEDSYFNIRLRGFWPYAEMQNKIEFKLKQYGIEIRKVAPNNTSKTCSKCGHLNNYFNFEYRKKNKFPHFKCEKCNFKENADYNAALNISNPKLKSTKEEPPKKKRKV

SEQ ID NO: 264 - protein, 529 aa, Artificial Sequence
  dCas12f1 R490L protein
MAKNTITKTLKLRIVRPYNSAEVEKIVADEKNNREKIALEKNKDKVKEACSKHLKVAAYCTTQVERNACLFCKARKLDDKFYQKLRGQFPDAVFWQEISEIFRQLQKQAAEIYNQSLIELYYEIFIKGKGIANASSVEHYLSDVCYTRAAELFKNAAIASGLRSKIKSNFRLKELKNMKSGLPTTKSDNFPIPLVKQKGGQYTGFEISNHNSDFIIKIPFGRWQVKKEIDKYRPWEKFDFEQVQKSPKPISLLLSTQRRKRNKGWSKDEGTEAEIKKVMNGDYQTSYIEVKRGSKIGEKSAWMLNLSIDVPKIDKGVDPSIIGGIDVGVKSPLVCAINNAFSRYSISDNDLFHFNKKMFARRRILLKKNRHKRAGHGAKNKLKPITILTEKSERFRKKLIERWACEIADFFIKNKVGTVQMENLESMKRKEDSYFNIRLRGFWPYAEMQNKIEFKLKQYGIEIRKVAPNNTSKTCSKCGHLNNYFNFEYLKKNKFPHFKCEKCNFKENADYNAALNISNPKLKSTKEEP

SEQ ID NO: 265 - protein, 529 aa, Artificial Sequence
  dCas12f1 R490W protein
MAKNTITKTLKLRIVRPYNSAEVEKIVADEKNNREKIALEKNKDKVKEACSKHLKVAAYCTTQVERNACLFCKARKLDDKFYQKLRGQFPDAVFWQEISEIFRQLQKQAAEIYNQSLIELYYEIFIKGKGIANASSVEHYLSDVCYTRAAELFKNAAIASGLRSKIKSNFRLKELKNMKSGLPTTKSDNFPIPLVKQKGGQYTGFEISNHNSDFIIKIPFGRWQVKKEIDKYRPWEKFDFEQVQKSPKPISLLLSTQRRKRNKGWSKDEGTEAEIKKVMNGDYQTSYIEVKRGSKIGEKSAWMLNLSIDVPKIDKGVDPSIIGGIDVGVKSPLVCAINNAFSRYSISDNDLFHFNKKMFARRRILLKKNRHKRAGHGAKNKLKPITILTEKSERFRKKLIERWACEIADFFIKNKVGTVQMENLESMKRKEDSYFNIRLRGFWPYAEMQNKIEFKLKQYGIEIRKVAPNNTSKTCSKCGHLNNYFNFEYWKKNKFPHFKCEKCNFKENADYNAALNISNPKLKSTKEEP

SEQ ID NO: 266 - protein, 529 aa, Artificial Sequence
  dCas12f1 D510A protein
MAKNTITKTLKLRIVRPYNSAEVEKIVADEKNNREKIALEKNKDKVKEACSKHLKVAAYCTTQVERNACLFCKARKLDDKFYQKLRGQFPDAVFWQEISEIFRQLQKQAAEIYNQSLIELYYEIFIKGKGIANASSVEHYLSDVCYTRAAELFKNAAIASGLRSKIKSNFRLKELKNMKSGLPTTKSDNFPIPLVKQKGGQYTGFEISNHNSDFIIKIPFGRWQVKKEIDKYRPWEKFDFEQVQKSPKPISLLLSTQRRKRNKGWSKDEGTEAEIKKVMNGDYQTSYIEVKRGSKIGEKSAWMLNLSIDVPKIDKGVDPSIIGGIDVGVKSPLVCAINNAFSRYSISDNDLFHFNKKMFARRRILLKKNRHKRAGHGAKNKLKPITILTEKSERFRKKLIERWACEIADFFIKNKVGTVQMENLESMKRKEDSYFNIRLRGFWPYAEMQNKIEFKLKQYGIEIRKVAPNNTSKTCSKCGHLNNYFNFEYRKKNKFPHFKCEKCNFKENAAYNAALNISNPKLKSTKEEP

SEQ ID NO: 267 - protein, 529 aa, Artificial Sequence
  dCas12f1 D510L protein
MAKNTITKTLKLRIVRPYNSAEVEKIVADEKNNREKIALEKNKDKVKEACSKHLKVAAYCTTQVERNACLFCKARKLDDKFYQKLRGQFPDAVFWQEISEIFRQLQKQAAEIYNQSLIELYYEIFIKGKGIANASSVEHYLSDVCYTRAAELFKNAAIASGLRSKIKSNFRLKELKNMKSGLPTTKSDNFPIPLVKQKGGQYTGFEISNHNSDFIIKIPFGRWQVKKEIDKYRPWEKFDFEQVQKSPKPISLLLSTQRRKRNKGWSKDEGTEAEIKKVMNGDYQTSYIEVKRGSKIGEKSAWMLNLSIDVPKIDKGVDPSIIGGIDVGVKSPLVCAINNAFSRYSISDNDLFHFNKKMFARRRILLKKNRHKRAGHGAKNKLKPITILTEKSERFRKKLIERWACEIADFFIKNKVGTVQMENLESMKRKEDSYFNIRLRGFWPYAEMQNKIEFKLKQYGIEIRKVAPNNTSKTCSKCGHLNNYFNFEYRKKNKFPHFKCEKCNFKENALYNAALNISNPKLKSTKEEP

SEQ ID NO: 268 - protein, 529 aa, Artificial Sequence
  dCas12f1 D510V protein
MAKNTITKTLKLRIVRPYNSAEVEKIVADEKNNREKIALEKNKDKVKEACSKHLKVAAYCTTQVERNACLFCKARKLDDKFYQKLRGQFPDAVFWQEISEIFRQLQKQAAEIYNQSLIELYYEIFIKGKGIANASSVEHYLSDVCYTRAAELFKNAAIASGLRSKIKSNFRLKELKNMKSGLPTTKSDNFPIPLVKQKGGQYTGFEISNHNSDFIIKIPFGRWQVKKEIDKYRPWEKFDFEQVQKSPKPISLLLSTQRRKRNKGWSKDEGTEAEIKKVMNGDYQTSYIEVKRGSKIGEKSAWMLNLSIDVPKIDKGVDPSIIGGIDVGVKSPLVCAINNAFSRYSISDNDLFHFNKKMFARRRILLKKNRHKRAGHGAKNKLKPITILTEKSERFRKKLIERWACEIADFFIKNKVGTVQMENLESMKRKEDSYFNIRLRGFWPYAEMQNKIEFKLKQYGIEIRKVAPNNTSKTCSKCGHLNNYFNFEYRKKNKFPHFKCEKCNFKENAVYNAALNISNPKLKSTKEEP

SEQ ID NO: 269 - protein, 529 aa, Artificial Sequence
  dCas12f1 E422A protein
MAKNTITKTLKLRIVRPYNSAEVEKIVADEKNNREKIALEKNKDKVKEACSKHLKVAAYCTTQVERNACLFCKARKLDDKFYQKLRGQFPDAVFWQEISEIFRQLQKQAAEIYNQSLIELYYEIFIKGKGIANASSVEHYLSDVCYTRAAELFKNAAIASGLRSKIKSNFRLKELKNMKSGLPTTKSDNFPIPLVKQKGGQYTGFEISNHNSDFIIKIPFGRWQVKKEIDKYRPWEKFDFEQVQKSPKPISLLLSTQRRKRNKGWSKDEGTEAEIKKVMNGDYQTSYIEVKRGSKIGEKSAWMLNLSIDVPKIDKGVDPSIIGGIDVGVKSPLVCAINNAFSRYSISDNDLFHFNKKMFARRRILLKKNRHKRAGHGAKNKLKPITILTEKSERFRKKLIERWACEIADFFIKNKVGTVQMANLESMKRKEDSYFNIRLRGFWPYAEMQNKIEFKLKQYGIEIRKVAPNNTSKTCSKCGHLNNYFNFEYRKKNKFPHFKCEKCNFKENADYNAALNISNPKLKSTKEEP

SEQ ID NO: 270 - DNA, 1586 bp, Artificial Sequence
  human codon-optimized Cas14a1
atggccaagaacacaattacaaagacactgaagctgaggatcgtgagaccatacaacagcgctgaggtcgagaagattgtggctgatgaaaagaacaacagggaaaagatcgccctcgagaagaacaaggataaggtgaaggaggcctgctctaagcacctgaaagtggccgcctactgcaccacacaggtggagaggaacgcctgtctgttttgtaaagctcggaagctggatgataagttttaccagaagctgcggggccagttccccgatgccgtcttttggcaggagattagcgagatcttcagacagctgcagaagcaggccgccgagatctacaaccagagcctgatcgagctctactacgagatcttcatcaagggcaagggcattgccaacgcctcctccgtggagcactacctgagcgacgtgtgctacacaagagccgccgagctctttaagaacgccgctatcgcttccgggctgaggagcaagattaagagtaacttccggctcaaggagctgaagaacatgaagagcggcctgcccactacaaagagcgacaacttcccaattccactggtgaagcagaaggggggccagtacacagggttcgagatttccaaccacaacagcgactttattattaagatcccctttggcaggtggcaggtcaagaaggagattgacaagtacaggccctgggagaagtttgatttcgagcaggtgcagaagagccccaagcctatttccctgctgctgtccacacagcggcggaagaggaacaaggggtggtctaaggatgaggggaccgaggccgagattaagaaagtgatgaacggcgactaccagacaagctacatcgaggtcaagcggggcagtaagattggcgagaagagcgcctggatgctgaacctgagcattgacgtgccaaagattgataagggcgtggatcccagcatcatcggagggatcgatgtgggggtcaagagccccctcgtgtgcgccatcaacaacgccttcagcaggtacagcatctccgataacgacctgttccactttaacaagaagatgttcgcccggcggaggattttgctcaagaagaaccggcacaagcgggccggacacggggccaagaacaagctcaagcccatcactatcctgaccgagaagagcgagaggttcaggaagaagctcatcgagagatgggcctgcgagatcgccgatttctttattaagaacaaggtcggaacagtgcagatggagaacctcgagagcatgaagaggaaggaggattcctacttcaacattcggctgagggggttctggccctacgctgagatgcagaacaagattgagtttaagctgaagcagtacgggattgagatccggaaggtggcccccaacaacaccagcaagacctgcagcaagtgcgggcacctcaacaactacttcaacttcgagtaccggaagaagaacaagttcccacacttcaagtgcgagaagtgcaactttaaggagaacgccgattacaacgccgccctgaacatcagcaaccctaagctgaagagcactaaggaggagcc

SEQ ID NO: 271 - protein, 529 aa, Artificial Sequence
  dCas12f1 D326A protein
MAKNTITKTLKLRIVRPYNSAEVEKIVADEKNNREKIALEKNKDKVKEACSKHLKVAAYCTTQVERNACLFCKARKLDDKFYQKLRGQFPDAVFWQEISEIFRQLQKQAAEIYNQSLIELYYEIFIKGKGIANASSVEHYLSDVCYTRAAELFKNAAIASGLRSKIKSNFRLKELKNMKSGLPTTKSDNFPIPLVKQKGGQYTGFEISNHNSDFIIKIPFGRWQVKKEIDKYRPWEKFDFEQVQKSPKPISLLLSTQRRKRNKGWSKDEGTEAEIKKVMNGDYQTSYIEVKRGSKIGEKSAWMLNLSIDVPKIDKGVDPSIIGGIAVGVKSPLVCAINNAFSRYSISDNDLFHFNKKMFARRRILLKKNRHKRAGHGAKNKLKPITILTEKSERFRKKLIERWACEIADFFIKNKVGTVQMENLESMKRKEDSYFNIRLRGFWPYAEMQNKIEFKLKQYGIEIRKVAPNNTSKTCSKCGHLNNYFNFEYRKKNKFPHFKCEKCNFKENADYNAALNISNPKLKSTKEEP

SEQ ID NO: 272 - protein, 51 aa, Artificial Sequence
  VP64 protein
MDALDDFDLDMLGSDALDDFDLDMLGSDALDDFDLDMLGSDALDDFDLDML

SEQ ID NO: 273 - DNA, 1628 bp, Artificial Sequence
  N/C-terminal NLS + Cas14a1 amino acid sequence
atgccaaagaagaagcggaaagtcgccaagaacacaattacaaagacactgaagctgaggatcgtgagaccatacaacagcgctgaggtcgagaagattgtggctgatgaaaagaacaacagggaaaagatcgccctcgagaagaacaaggataaggtgaaggaggcctgctctaagcacctgaaagtggccgcctactgcaccacacaggtggagaggaacgcctgtctgttttgtaaagctcggaagctggatgataagttttaccagaagctgcggggccagttccccgatgccgtcttttggcaggagattagcgagatcttcagacagctgcagaagcaggccgccgagatctacaaccagagcctgatcgagctctactacgagatcttcatcaagggcaagggcattgccaacgcctcctccgtggagcactacctgagcgacgtgtgctacacaagagccgccgagctctttaagaacgccgctatcgcttccgggctgaggagcaagattaagagtaacttccggctcaaggagctgaagaacatgaagagcggcctgcccactacaaagagcgacaacttcccaattccactggtgaagcagaaggggggccagtacacagggttcgagatttccaaccacaacagcgactttattattaagatcccctttggcaggtggcaggtcaagaaggagattgacaagtacaggccctgggagaagtttgatttcgagcaggtgcagaagagccccaagcctatttccctgctgctgtccacacagcggcggaagaggaacaaggggtggtctaaggatgaggggaccgaggccgagattaagaaagtgatgaacggcgactaccagacaagctacatcgaggtcaagcggggcagtaagattggcgagaagagcgcctggatgctgaacctgagcattgacgtgccaaagattgataagggcgtggatcccagcatcatcggagggatcgatgtgggggtcaagagccccctcgtgtgcgccatcaacaacgccttcagcaggtacagcatctccgataacgacctgttccactttaacaagaagatgttcgcccggcggaggattttgctcaagaagaaccggcacaagcgggccggacacggggccaagaacaagctcaagcccatcactatcctgaccgagaagagcgagaggttcaggaagaagctcatcgagagatgggcctgcgagatcgccgatttctttattaagaacaaggtcggaacagtgcagatggagaacctcgagagcatgaagaggaaggaggattcctacttcaacattcggctgagggggttctggccctacgctgagatgcagaacaagattgagtttaagctgaagcagtacgggattgagatccggaaggtggcccccaacaacaccagcaagacctgcagcaagtgcgggcacctcaacaactacttcaacttcgagtaccggaagaagaacaagttcccacacttcaagtgcgagaagtgcaactttaaggagaacgccgattacaacgccgccctgaacatcagcaaccctaagctgaagagcactaaggaggagccccaaagaagaagcggaaagtc

SEQ ID NO: 274 - protein, 65 aa, Artificial Sequence
  KRAB amino acids sequence
RTLVTFKDVFVDFTREEWKLLDTAQQIVYRNVMLENYKNLVSLGYQLTKPDVILRLEKGEEPWLV

SEQ ID NO: 275 - protein, 286 aa, Artificial Sequence
  MeCP2 amino acids sequence
VQVKRVLEKSPGKLLVKMPFQASPGGKGEGGGATTSAQVMVIKRPGRKRKAEADPQAIPKKRGRKPGSVVAAAAAEAKKKAVKESSIRSVQETVLPIKKRKTRETVSIEVKEVVKPLLVSTLGEKSGKGLKTCKSPGRKSKESSPKGRSSSASSPPKKEHHHHHHHAESPKAPMPLLPPPPPPEPQSSEDPISPPEPQDLSSSICKEEKMPRAGSLESDGCPKEPAKTQPMVAAAATTTTTTTTTVAEKYKHRGEGERKDIVSSSMPRPNREEPVDSRTPVTERVS

SEQ ID NO: 276 - protein, 311 aa, Artificial Sequence
  DNMT3A amino acids sequence
PSRLQMFFANNHDQEFDPPKVYPPVPAEKRKPIRVLSLFDGIATGLLVLKDLGIQVDRYIASEVCEDSITVGMVRHQGKIMYVGDVRSVTQKHIQEWGPFDLVIGGSPCNDLSIVNPARKGLYEGTGRLFFEFYRLLHDARPKEGDDRPFFWLFENVVAMGVSDKRDISRFLESNPVMIDAKEVSAAHRARYFWGNLPGMNRPLASTVNDKLELQECLEHGRIAKFSKVRTITTRSNSIKQGKDQHFPVFMNEKEDILWCTEMERVFGFPVHYTDVSNMSRLARQRLLGRSWSVPVIRHLFAPLKEYFACV

SEQ ID NO: 277 - protein, 428 aa, Artificial Sequence
  HDAC3 amino acids sequence
MAKTVAYFYDPDVGNFHYGAGHPMKPHRLALTHSLVLHYGLYKKMIVFKPYQASQHDMCRFHSEDYIDFLQRVSPTNMQGFTKSLNAFNVGDDCPVFPGLFEFCSRYTGASLQGATQLNNKICDIAINWAGGLHHAKKFEASGFCYVNDIVIGILELLKYHPRVLYIDIDIHHGDGVQEAFYLTDRVMTVSFHKYGNYFFPGTGDMYEVGAESGRYYCLNVPLRDGIDDQSYKHLFQPVINQVVDFYQPTCIVLQCGADSLGCDRLGCFNLSIRGHGECVEYVKSFNIPLLVLGGGGYTVRNVARCWTYETSLLVEEAISEELPYSEYFEYFAPDFTLHPDVSTRIENQNSRQYLDQIRQTIFENLKMLNHAPSVQIHDVPADLLTYDRTDEADAEERGPEENYSRPEAPNEFYDGDHDNDKESDVEI

SEQ ID NO: 278 - protein, 7 aa, simian virus 40
PKKKRKV

SEQ ID NO: 279 - protein, 16 aa, mus musculus
KRPAATKKAGQAKKKK

SEQ ID NO: 280 - protein, 9 aa, homo sapiens
PAAKRVKLD

SEQ ID NO: 281 - protein, 11 aa, Homo sapiens
RQRRNELKRSP

SEQ ID NO: 282 - protein, 38 aa, mus musculus
NQSSNFGPMKGGNFGGRSSGPYGGGGQYFAKPRNQGGY

SEQ ID NO: 283 - protein, 42 aa, Homo sapiens
RMRIZFKNKGKDTAELRRRRVEVSVELRKAKKDEQILKRRNV

SEQ ID NO: 284 - protein, 8 aa, Homo sapiens
VSRKRPRP

SEQ ID NO: 285 - protein, 8 aa, homo sapiens
PPKKARED

SEQ ID NO: 286 - protein, 8 aa, homo sapiens
PQPKKKPL

SEQ ID NO: 287 - protein, 12 aa, mus musculus
SALIKKKKKMAP

SEQ ID NO: 288 - protein, 5 aa, Influenza virus
DRLRR

SEQ ID NO: 289 - protein, 7 aa, influenza virus
PKQKKRK

SEQ ID NO: 290 - protein, 10 aa, Hepatitis D virus
RKLKKKIKKL

SEQ ID NO: 291 - protein, 10 aa, mus musculus
REKKKFLKRR

SEQ ID NO: 292 - protein, 20 aa, homo sapiens
KRKGDEVDGVDEVAKKKSKK

SEQ ID NO: 293 - protein, 17 aa, Homo sapiens
RKCLQAGMNLEARKTKK

SEQ ID NO: 294 - RNA, 181 nt, Artificial Sequence
  Comperative Example 1.1.1
cuucacugauaaaguggagaaccgcuucaccaaaagcugucccuuaggggauuagaacuugagugaaggugggcugcuugcaucagccuaaugucgagaagugcuuucuucggaaaguaacccucgaaacaaauucauuugaaagaaugaaggaaugcaaccacacacacagugggcuacc

SEQ ID NO: 295 - RNA, 190 nt, Artificial Sequence
  Comperative Example 1.1.2
cuucacugauaaaguggagaaccgcuucaccaaaagcugucccuuaggggauuagaacuugagugaaggugggcugcuugcaucagccuaaugucgagaagugcuuucuucggaaaguaacccucgaaacaaauucauuugaaagaaugaaggaaugcaaccacacacacagugggcuaccuuuuauuuu

SEQ ID NO: 296 - RNA, 183 nt, Artificial Sequence
  Example 1.1.1
gauaaaguggagaaccgcuucaccaaaagcugucccuuaggggauuagaacuugagugaaggugggcugcuugcaucagccuaaugucgagaagugcuuucuucggaaaguaacccucgaaacaaauucauuugaaagaaugaaggaaugcaaccacacacacagugggcuaccuuuuauuuu

SEQ ID NO: 297 - RNA, 176 nt, Artificial Sequence
  Example 1.1.2
uggagaaccgcuucaccaaaagcugucccuuaggggauuagaacuugagugaaggugggcugcuugcaucagccuaaugucgagaagugcuuucuucggaaaguaacccucgaaacaaauucauuugaaagaaugaaggaaugcaaccacacacacagugggcuaccuuuuauuuu

SEQ ID NO: 298 - RNA, 170 nt, Artificial Sequence
  Example 1.1.3
accgcuucaccaaaagcugucccuuaggggauuagaacuugagugaaggugggcugcuugcaucagccuaaugucgagaagugcuuucuucggaaaguaacccucgaaacaaauucauuugaaagaaugaaggaaugcaaccacacacacagugggcuaccuuuuauuuu

SEQ ID NO: 299 - RNA, 184 nt, Artificial Sequence
  Example 1.1.4
cuucacugauaaaguggagaaccgcuucaccaaaagcuguuuagauuagaacuugagugaaggugggcugcuugcaucagccuaaugucgagaagugcuuucuucggaaaguaacccucgaaacaaauucauuugaaagaaugaaggaaugcaaccacacacacagugggcuaccuuuuauuuu

SEQ ID NO: 300 - RNA, 179 nt, Artificial Sequence
  Example 1.1.5
cuucacugauaaaguggagaaccgcuucaccaaaagcuuuagagaacuugagugaaggugggcugcuugcaucagccuaaugucgagaagugcuuucuucggaaaguaacccucgaaacaaauucauuugaaagaaugaaggaaugcaaccacacacacagugggcuaccuuuuauuuu

SEQ ID NO: 301 - RNA, 169 nt, Artificial Sequence
  Example 1.1.6
cuucacugauaaaguggagaaccgcuucaccaauuaguugagugaaggugggcugcuugcaucagccuaaugucgagaagugcuuucuucggaaaguaacccucgaaacaaauucauuugaaagaaugaaggaaugcaaccacacacacagugggcuaccuuuuauuuu

SEQ ID NO: 302 - RNA, 186 nt, Artificial Sequence
  Example 1.1.7
cuucacugauaaaguggagaaccgcuucaccaaaagcugucccuuaggggauuagaacuugagugaaggugggcugcuugcaucagccuaaugucgagaagugcuuucuucggaaaguaacccucgaaacaaauucaugaaaaugaaggaaugcaaccacacacacagugggcuaccuuuuauuuu

SEQ ID NO: 303 - RNA, 182 nt, Artificial Sequence
  Example 1.1.8
cuucacugauaaaguggagaaccgcuucaccaaaagcugucccuuaggggauuagaacuugagugaaggugggcugcuugcaucagccuaaugucgagaagugcuuucuucggaaaguaacccucgaaacaaauucgaaagaaggaaugcaaccacacacacagugggcuaccuuuuauuuu

SEQ ID NO: 304 - RNA, 176 nt, Artificial Sequence
  Example 1.1.9
cuucacugauaaaguggagaaccgcuucaccaaaagcugucccuuaggggauuagaacuugagugaaggugggcugcuugcaucagccuaaugucgagaagugcuuucuucggaaaguaacccucgaaacaaagaaaggaaugcaaccacacacacagugggcuaccuuuuauuuu

SEQ ID NO: 305 - RNA, 147 nt, Artificial Sequence
  Example 1.1.10
accgcuucaccauuagugagugaaggugggcugcuugcaucagccuaaugucgagaagugcuuucuucggaaaguaacccucgaaacaaauucauuugaaagaaugaaggaaugcaaccacacacacagugggcuaccuuuuauuuu

SEQ ID NO: 306 - RNA, 156 nt, Artificial Sequence
  Example 1.1.11
accgcuucaccaaaagcugucccuuaggggauuagaacuugagugaaggugggcugcuugcaucagccuaaugucgagaagugcuuucuucggaaaguaacccucgaaacaaagaaaggaaugcaaccacacacacagugggcuaccuuuuauuuu

SEQ ID NO: 307 - RNA, 153 nt, Artificial Sequence
  Example 1.1.12
cuucacugauaaaguggagaaccgcuucaccauuagugagugaaggugggcugcuugcaucagccuaaugucgagaagugcuuucuucggaaaguaacccucgaaacaaagaaaggaaugcaaccacacacacagugggcuaccuuuuauuuu

SEQ ID NO: 308 - RNA, 133 nt, Artificial Sequence
  Example 1.1.13
accgcuucaccauuagugagugaaggugggcugcuugcaucagccuaaugucgagaagugcuuucuucggaaaguaacccucgaaacaaagaaaggaaugcaaccacacacacagugggcuaccuuuuauuuu

SEQ ID NO: 309 - RNA, 181 nt, Artificial Sequence
  Comperative Example 1.2.1
cuucacugauaaaguggagaaccgcuucaccaaaagcugucccuuaggggauuagaacuugagugaaggugggcugcuugcaucagccuaaugucgagaagugcuuucuucggaaaguaacccucgaaacaaauucauuugaaagaaugaaggaaugcaaccauccccaggacacacacac

SEQ ID NO: 310 - RNA, 190 nt, Artificial Sequence
  Comperative Example 1.2.2
cuucacugauaaaguggagaaccgcuucaccaaaagcugucccuuaggggauuagaacuugagugaaggugggcugcuugcaucagccuaaugucgagaagugcuuucuucggaaaguaacccucgaaacaaauucauuugaaagaaugaaggaaugcaaccauccccaggacacacacacuuuuauuuu

SEQ ID NO: 311 - RNA, 183 nt, Artificial Sequence
  Example 1.2.1
gauaaaguggagaaccgcuucaccaaaagcugucccuuaggggauuagaacuugagugaaggugggcugcuugcaucagccuaaugucgagaagugcuuucuucggaaaguaacccucgaaacaaauucauuugaaagaaugaaggaaugcaaccauccccaggacacacacacuuuuauuuu

SEQ ID NO: 312 - RNA, 176 nt, Artificial Sequence
  Example 1.2.2
uggagaaccgcuucaccaaaagcugucccuuaggggauuagaacuugagugaaggugggcugcuugcaucagccuaaugucgagaagugcuuucuucggaaaguaacccucgaaacaaauucauuugaaagaaugaaggaaugcaaccauccccaggacacacacacuuuuauuuu

SEQ ID NO: 313 - RNA, 170 nt, Artificial Sequence
  Example 1.2.3
accgcuucaccaaaagcugucccuuaggggauuagaacuugagugaaggugggcugcuugcaucagccuaaugucgagaagugcuuucuucggaaaguaacccucgaaacaaauucauuugaaagaaugaaggaaugcaaccauccccaggacacacacacuuuuauuuu

SEQ ID NO: 314 - RNA, 184 nt, Artificial Sequence
  Example 1.2.4
cuucacugauaaaguggagaaccgcuucaccaaaagcuguuuagauuagaacuugagugaaggugggcugcuugcaucagccuaaugucgagaagugcuuucuucggaaaguaacccucgaaacaaauucauuugaaagaaugaaggaaugcaaccauccccaggacacacacacuuuuauuuu

SEQ ID NO: 315 - RNA, 178 nt, Artificial Sequence
  Example 1.2.5
cuucacugauaaaguggagaaccgcuucaccaaaagcuuagagaacuugagugaaggugggcugcuugcaucagccuaaugucgagaagugcuuucuucggaaaguaacccucgaaacaaauucauuugaaagaaugaaggaaugcaaccauccccaggacacacacacuuuuauuuu

SEQ ID NO: 316 - RNA, 167 nt, Artificial Sequence
  Example 1.2.6
cuucacugauaaaguggagaaccgcuucaccauuagugagugaaggugggcugcuugcaucagccuaaugucgagaagugcuuucuucggaaaguaacccucgaaacaaauucauuugaaagaaugaaggaaugcaaccauccccaggacacacacacuuuuauuuu

SEQ ID NO: 317 - RNA, 186 nt, Artificial Sequence
  Example 1.2.7
cuucacugauaaaguggagaaccgcuucaccaaaagcugucccuuaggggauuagaacuugagugaaggugggcugcuugcaucagccuaaugucgagaagugcuuucuucggaaaguaacccucgaaacaaauucaugaaaaugaaggaaugcaaccauccccaggacacacacacuuuuauuuu

SEQ ID NO: 318 - RNA, 182 nt, Artificial Sequence
  Example 1.2.8
cuucacugauaaaguggagaaccgcuucaccaaaagcugucccuuaggggauuagaacuugagugaaggugggcugcuugcaucagccuaaugucgagaagugcuuucuucggaaaguaacccucgaaacaaauucgaaagaaggaaugcaaccauccccaggacacacacacuuuuauuuu

SEQ ID NO: 319 - RNA, 176 nt, Artificial Sequence
  Example 1.2.9
cuucacugauaaaguggagaaccgcuucaccaaaagcugucccuuaggggauuagaacuugagugaaggugggcugcuugcaucagccuaaugucgagaagugcuuucuucggaaaguaacccucgaaacaaagaaaggaaugcaaccauccccaggacacacacacuuuuauuuu

SEQ ID NO: 320 - RNA, 147 nt, Artificial Sequence
  Example 1.2.10
accgcuucaccauuagugagugaaggugggcugcuugcaucagccuaaugucgagaagugcuuucuucggaaaguaacccucgaaacaaauucauuugaaagaaugaaggaaugcaaccauccccaggacacacacacuuuuauuuu

SEQ ID NO: 321 - RNA, 156 nt, Artificial Sequence
  Example 1.2.11
accgcuucaccaaaagcugucccuuaggggauuagaacuugagugaaggugggcugcuugcaucagccuaaugucgagaagugcuuucuucggaaaguaacccucgaaacaaagaaaggaaugcaaccauccccaggacacacacacuuuuauuuu

SEQ ID NO: 322 - RNA, 153 nt, Artificial Sequence
  Example 1.2.12
cuucacugauaaaguggagaaccgcuucaccauuagugagugaaggugggcugcuugcaucagccuaaugucgagaagugcuuucuucggaaaguaacccucgaaacaaagaaaggaaugcaaccauccccaggacacacacacuuuuauuuu

SEQ ID NO: 323 - RNA, 133 nt, Artificial Sequence
  Example 1.2.13
accgcuucaccauuagugagugaaggugggcugcuugcaucagccuaaugucgagaagugcuuucuucggaaaguaacccucgaaacaaagaaaggaaugcaaccauccccaggacacacacacuuuuauuuu

SEQ ID NO: 324 - RNA, 181 nt, Artificial Sequence
  Comperative Example 1.3.1
cuucacugauaaaguggagaaccgcuucaccaaaagcugucccuuaggggauuagaacuugagugaaggugggcugcuugcaucagccuaaugucgagaagugcuuucuucggaaaguaacccucgaaacaaauucauuugaaagaaugaaggaaugcaacagaacacauaccccugggcc

SEQ ID NO: 325 - RNA, 190 nt, Artificial Sequence
  Comperative Example 1.3.2
cuucacugauaaaguggagaaccgcuucaccaaaagcugucccuuaggggauuagaacuugagugaaggugggcugcuugcaucagccuaaugucgagaagugcuuucuucggaaaguaacccucgaaacaaauucauuugaaagaaugaaggaaugcaacagaacacauaccccugggccuuuuauuuu

SEQ ID NO: 326 - RNA, 183 nt, Artificial Sequence
  Example 1.3.1
gauaaaguggagaaccgcuucaccaaaagcugucccuuaggggauuagaacuugagugaaggugggcugcuugcaucagccuaaugucgagaagugcuuucuucggaaaguaacccucgaaacaaauucauuugaaagaaugaaggaaugcaacagaacacauaccccugggccuuuuauuuu

SEQ ID NO: 327 - RNA, 176 nt, Artificial Sequence
  Example 1.3.2
uggagaaccgcuucaccaaaagcugucccuuaggggauuagaacuugagugaaggugggcugcuugcaucagccuaaugucgagaagugcuuucuucggaaaguaacccucgaaacaaauucauuugaaagaaugaaggaaugcaacagaacacauaccccugggccuuuuauuuu

SEQ ID NO: 328 - RNA, 170 nt, Artificial Sequence
  Example 1.3.3
accgcuucaccaaaagcugucccuuaggggauuagaacuugagugaaggugggcugcuugcaucagccuaaugucgagaagugcuuucuucggaaaguaacccucgaaacaaauucauuugaaagaaugaaggaaugcaacagaacacauaccccugggccuuuuauuuu

SEQ ID NO: 329 - RNA, 184 nt, Artificial Sequence
  Example 1.3.4
cuucacugauaaaguggagaaccgcuucaccaaaagcuguuuagauuagaacuugagugaaggugggcugcuugcaucagccuaaugucgagaagugcuuucuucggaaaguaacccucgaaacaaauucauuugaaagaaugaaggaaugcaacagaacacauaccccugggccuuuuauuuu

SEQ ID NO: 330 - RNA, 179 nt, Artificial Sequence
  Example 1.3.5
cuucacugauaaaguggagaaccgcuucaccaaaagcuuuagagaacuugagugaaggugggcugcuugcaucagccuaaugucgagaagugcuuucuucggaaaguaacccucgaaacaaauucauuugaaagaaugaaggaaugcaacagaacacauaccccugggccuuuuauuuu

SEQ ID NO: 331 - RNA, 169 nt, Artificial Sequence
  Example 1.3.6
cuucacugauaaaguggagaaccgcuucaccaauuaguugagugaaggugggcugcuugcaucagccuaaugucgagaagugcuuucuucggaaaguaacccucgaaacaaauucauuugaaagaaugaaggaaugcaacagaacacauaccccugggccuuuuauuuu

SEQ ID NO: 332 - RNA, 186 nt, Artificial Sequence
  Example 1.3.7
cuucacugauaaaguggagaaccgcuucaccaaaagcugucccuuaggggauuagaacuugagugaaggugggcugcuugcaucagccuaaugucgagaagugcuuucuucggaaaguaacccucgaaacaaauucaugaaaaugaaggaaugcaacagaacacauaccccugggccuuuuauuuu

SEQ ID NO: 333 - RNA, 182 nt, Artificial Sequence
  Example 1.3.8
cuucacugauaaaguggagaaccgcuucaccaaaagcugucccuuaggggauuagaacuugagugaaggugggcugcuugcaucagccuaaugucgagaagugcuuucuucggaaaguaacccucgaaacaaauucgaaagaaggaaugcaacagaacacauaccccugggccuuuuauuuu

SEQ ID NO: 334 - RNA, 176 nt, Artificial Sequence
  Example 1.3.9
cuucacugauaaaguggagaaccgcuucaccaaaagcugucccuuaggggauuagaacuugagugaaggugggcugcuugcaucagccuaaugucgagaagugcuuucuucggaaaguaacccucgaaacaaagaaaggaaugcaacagaacacauaccccugggccuuuuauuuu

SEQ ID NO: 335 - RNA, 147 nt, Artificial Sequence
  Example 1.3.10
accgcuucaccauuagugagugaaggugggcugcuugcaucagccuaaugucgagaagugcuuucuucggaaaguaacccucgaaacaaauucauuugaaagaaugaaggaaugcaacagaacacauaccccugggccuuuuauuuu

SEQ ID NO: 336 - RNA, 156 nt, Artificial Sequence
  Example 1.3.11
accgcuucaccaaaagcugucccuuaggggauuagaacuugagugaaggugggcugcuugcaucagccuaaugucgagaagugcuuucuucggaaaguaacccucgaaacaaagaaaggaaugcaacagaacacauaccccugggccuuuuauuuu

SEQ ID NO: 337 - RNA, 153 nt, Artificial Sequence
  Example 1.3.12
cuucacugauaaaguggagaaccgcuucaccauuagugagugaaggugggcugcuugcaucagccuaaugucgagaagugcuuucuucggaaaguaacccucgaaacaaagaaaggaaugcaacagaacacauaccccugggccuuuuauuuu

SEQ ID NO: 338 - RNA, 133 nt, Artificial Sequence
  Example 1.3.13
accgcuucaccauuagugagugaaggugggcugcuugcaucagccuaaugucgagaagugcuuucuucggaaaguaacccucgaaacaaagaaaggaaugcaacagaacacauaccccugggccuuuuauuuu

SEQ ID NO: 339 - DNA, 20 bp, Artificial Sequence
  Protospacer sequence for targeting DY2
cacacacacagtgggctacc

SEQ ID NO: 340 - DNA, 20 bp, Artificial Sequence
  Protospacer sequence for targeting DY10
catccccaggacacacacac

SEQ ID NO: 341 - DNA, 20 bp, Artificial Sequence
  Protospacer sequence for targeting Intergenic-22
agaacacatacccctgggcc

SEQ ID NO: 342 - RNA, 23 nt, Artificial Sequence
  modified second region
ccgcuucacuuaggugaaggugg

SEQ ID NO: 343 - RNA, 11 nt, Artificial Sequence
  modified second region
ccguuaggugg

SEQ ID NO: 344 - RNA, 13 nt, Artificial Sequence
  modified second region
ccgcuuagggugg

SEQ ID NO: 345 - RNA, 15 nt, Artificial Sequence
  modified second region
ccgcuuuagaggugg

SEQ ID NO: 346 - RNA, 17 nt, Artificial Sequence
  modified second region
ccgcuuuuagaaggugg

SEQ ID NO: 347 - RNA, 19 nt, Artificial Sequence
  modified second region
ccgcuucuuaggaaggugg

SEQ ID NO: 348 - RNA, 21 nt, Artificial Sequence
  modified second region
ccgcuucauuagugaaggugg

SEQ ID NO: 349 - RNA, 23 nt, Artificial Sequence
  modified second region
ccgcuucacuuaggugaaggugg

SEQ ID NO: 350 - RNA, 24 nt, Artificial Sequence
  modified second region
ccgcuucacuuagagugaaggugg

SEQ ID NO: 351 - RNA, 26 nt, Artificial Sequence
  modified second region
ccgcuucaccuuaggagugaaggugg

SEQ ID NO: 352 - RNA, 28 nt, Artificial Sequence
  modified second region
ccgcuucaccauuagugagugaaggugg

SEQ ID NO: 353 - RNA, 30 nt, Artificial Sequence; identical to SEQ ID NO: 40
  modified second region

SEQ ID NO: 354 - RNA, 32 nt, Artificial Sequence; identical to SEQ ID NO: 41
  modified second region

SEQ ID NO: 355 - RNA, 34 nt, Artificial Sequence; identical to SEQ ID NO: 42
  modified second region

SEQ ID NO: 356 - RNA, 36 nt, Artificial Sequence; identical to SEQ ID NO: 43
  modified second region

SEQ ID NO: 357 - RNA, 38 nt, Artificial Sequence; identical to SEQ ID NO: 44
  modified second region

SEQ ID NO: 358 - RNA, 40 nt, Artificial Sequence; identical to SEQ ID NO: 45
  modified second region

SEQ ID NO: 359 - RNA, 42 nt, Artificial Sequence; identical to SEQ ID NO: 47
  modified second region

SEQ ID NO: 360 - RNA, 43 nt, Artificial Sequence; identical to SEQ ID NO: 46
  modified second region

SEQ ID NO: 361 - RNA, 45 nt, Artificial Sequence; identical to SEQ ID NO: 48
  modified second region

SEQ ID NO: 362 - RNA, 47 nt, Artificial Sequence; identical to SEQ ID NO: 49
  modified second region

SEQ ID NO: 363 - RNA, 10 nt, Artificial Sequence
  modified second region, upper part (5' to UUAG)
ccgcuuuuag

SEQ ID NO: 364 - RNA, 11 nt, Artificial Sequence
  modified second region, upper part (5' to UUAG)
ccgcuucuuag

SEQ ID NO: 365 - RNA, 12 nt, Artificial Sequence
  modified second region, upper part (5' to UUAG)
ccgcuucauuag

SEQ ID NO: 366 - RNA, 13 nt, Artificial Sequence
  modified second region, upper part (5' to UUAG)
ccgcuucacuuag

SEQ ID NO: 367 - RNA, 14 nt, Artificial Sequence
  modified second region, upper part (5' to UUAG)
ccgcuucaccuuag

SEQ ID NO: 368 - RNA, 15 nt, Artificial Sequence
  modified second region, upper part (5' to UUAG)
ccgcuucaccauuag

SEQ ID NO: 369 - RNA, 16 nt, Artificial Sequence
  modified second region, upper part (5' to UUAG)
ccgcuucaccaauuag

SEQ ID NO: 370 - RNA, 17 nt, Artificial Sequence
  modified second region, upper part (5' to UUAG)
ccgcuucaccaaauuag

SEQ ID NO: 371 - RNA, 18 nt, Artificial Sequence
  modified second region, upper part (5' to UUAG)
ccgcuucaccaaaauuag

SEQ ID NO: 372 - RNA, 19 nt, Artificial Sequence
  modified second region, upper part (5' to UUAG)
ccgcuucaccaaaaguuag

SEQ ID NO: 373 - RNA, 20 nt, Artificial Sequence
  modified second region, upper part (5' to UUAG)
ccgcuucaccaaaagcuuag

SEQ ID NO: 374 - RNA, 21 nt, Artificial Sequence
  modified second region, upper part (5' to UUAG)
ccgcuucaccaaaagcuuuag

SEQ ID NO: 375 - RNA, 22 nt, Artificial Sequence
  modified second region, upper part (5' to UUAG)
ccgcuucaccaaaagcuguuag

SEQ ID NO: 376 - RNA, 23 nt, Artificial Sequence
  modified second region, upper part (5' to UUAG)
ccgcuucaccaaaagcuguuuag

SEQ ID NO: 377 - RNA, 24 nt, Artificial Sequence
  modified second region, upper part (5' to UUAG)
ccgcuucaccaaaagcugucuuag

SEQ ID NO: 378 - RNA, 25 nt, Artificial Sequence
  modified second region, upper part (5' to UUAG)
ccgcuucaccaaaagcuguccuuag

SEQ ID NO: 379 - RNA, 119 nt, Artificial Sequence
  engineered tracrRNA(mature form, the first region is deleted)
ccgcuucaccaaaagcugucccuuaggggauuagaacuugagugaaggugggcugcuugcaucagccuaaugucgagaagugcuuucuucggaaaguaacccucgaaacaaauucauuu

SEQ ID NO: 380 - RNA, 89 nt, Artificial Sequence
  engineered tracrRNA(mature form, the second region is deleted)
cuucacugauaaaguggagaagcugcuugcaucagccuaaugucgagaagugcuuucuucggaaaguaacccucgaaacaaauucauuu

SEQ ID NO: 381 - RNA, 90 nt, Artificial Sequence
  engineered tracrRNA(mature form, having modified second region)
cuucacugauaaaguggagaaggcugcuugcaucagccuaaugucgagaagugcuuucuucggaaaguaacccucgaaacaaauucauuu

SEQ ID NO: 382 - RNA, 94 nt, Artificial Sequence
  engineered tracrRNA(mature form, having modified second region)
cuucacugauaaaguggagaauuagggcugcuugcaucagccuaaugucgagaagugcuuucuucggaaaguaacccucgaaacaaauucauuu

SEQ ID NO: 383 - RNA, 96 nt, Artificial Sequence
  engineered tracrRNA(mature form, having modified second region)
cuucacugauaaaguggagaacuuaggggcugcuugcaucagccuaaugucgagaagugcuuucuucggaaaguaacccucgaaacaaauucauuu

SEQ ID NO: 384 - RNA, 97 nt, Artificial Sequence
  engineered tracrRNA(mature form, having modified second region)
cuucacugauaaaguggagaacuuagugggcugcuugcaucagccuaaugucgagaagugcuuucuucggaaaguaacccucgaaacaaauucauuu

SEQ ID NO: 385 - RNA, 99 nt, Artificial Sequence
  engineered tracrRNA(mature form, having modified second region)
cuucacugauaaaguggagaaccuuaggugggcugcuugcaucagccuaaugucgagaagugcuuucuucggaaaguaacccucgaaacaaauucauuu

SEQ ID NO: 386 - RNA, 100 nt, Artificial Sequence
  engineered tracrRNA(mature form, having modified second region)
cuucacugauaaaguggagaaccguuaggugggcugcuugcaucagccuaaugucgagaagugcuuucuucggaaaguaacccucgaaacaaauucauuu

SEQ ID NO: 387 - RNA, 102 nt, Artificial Sequence
  engineered tracrRNA(mature form, having modified second region)
cuucacugauaaaguggagaaccgcuuagggugggcugcuugcaucagccuaaugucgagaagugcuuucuucggaaaguaacccucgaaacaaauucauuu

SEQ ID NO: 388 - RNA, 104 nt, Artificial Sequence
  engineered tracrRNA(mature form, having modified second region)
cuucacugauaaaguggagaaccgcuuuagaggugggcugcuugcaucagccuaaugucgagaagugcuuucuucggaaaguaacccucgaaacaaauucauuu

SEQ ID NO: 389 - RNA, 106 nt, Artificial Sequence
  engineered tracrRNA(mature form, having modified second region)
cuucacugauaaaguggagaaccgcuuuuagaaggugggcugcuugcaucagccuaaugucgagaagugcuuucuucggaaaguaacccucgaaacaaauucauuu

SEQ ID NO: 390 - RNA, 108 nt, Artificial Sequence
  engineered tracrRNA(mature form, having modified second region)
cuucacugauaaaguggagaaccgcuucuuaggaaggugggcugcuugcaucagccuaaugucgagaagugcuuucuucggaaaguaacccucgaaacaaauucauuu

SEQ ID NO: 391 - RNA, 110 nt, Artificial Sequence
  engineered tracrRNA(mature form, having modified second region)
cuucacugauaaaguggagaaccgcuucauuagugaaggugggcugcuugcaucagccuaaugucgagaagugcuuucuucggaaaguaacccucgaaacaaauucauuu

SEQ ID NO: 392 - RNA, 112 nt, Artificial Sequence
  engineered tracrRNA(mature form, having modified second region)
cuucacugauaaaguggagaaccgcuucacuuaggugaaggugggcugcuugcaucagccuaaugucgagaagugcuuucuucggaaaguaacccucgaaacaaauucauuu

SEQ ID NO: 393 - RNA, 113 nt, Artificial Sequence
  engineered tracrRNA(mature form, having modified second region)
cuucacugauaaaguggagaaccgcuucacuuagagugaaggugggcugcuugcaucagccuaaugucgagaagugcuuucuucggaaaguaacccucgaaacaaauucauuu

SEQ ID NO: 394 - RNA, 115 nt, Artificial Sequence
  engineered tracrRNA(mature form, having modified second region)
cuucacugauaaaguggagaaccgcuucaccuuaggagugaaggugggcugcuugcaucagccuaaugucgagaagugcuuucuucggaaaguaacccucgaaacaaauucauuu

SEQ ID NO: 395 - RNA, 117 nt, Artificial Sequence; identical to SEQ ID NO: 139
  engineered tracrRNA(mature form, having modified second region)

SEQ ID NO: 396 - RNA, 119 nt, Artificial Sequence; identical to SEQ ID NO: 140
  engineered tracrRNA(mature form, having modified second region)

SEQ ID NO: 397 - RNA, 121 nt, Artificial Sequence
  engineered tracrRNA(mature form, having modified second region)
cuucacugauaaaguggagaaccgcuucaccaaauuagcuugagugaaggugggcugcuugcaucagccuaaugucgagaagugcuuucuucggaaaguaacccucgaaacaaauucauuu

SEQ ID NO: 398 - RNA, 123 nt, Artificial Sequence
  engineered tracrRNA(mature form, having modified second region)
cuucacugauaaaguggagaaccgcuucaccaaaauuagacuugagugaaggugggcugcuugcaucagccuaaugucgagaagugcuuucuucggaaaguaacccucgaaacaaauucauuu

SEQ ID NO: 399 - RNA, 125 nt, Artificial Sequence; identical to SEQ ID NO: 142
  engineered tracrRNA(mature form, having modified second region)

SEQ ID NO: 400 - RNA, 127 nt, Artificial Sequence; identical to SEQ ID NO: 143
  engineered tracrRNA(mature form, having modified second region)

SEQ ID NO: 401 - RNA, 129 nt, Artificial Sequence; identical to SEQ ID NO: 144
  engineered tracrRNA(mature form, having modified second region)

SEQ ID NO: 402 - RNA, 131 nt, Artificial Sequence; identical to SEQ ID NO: 146
  engineered tracrRNA(mature form, having modified second region)

SEQ ID NO: 403 - RNA, 132 nt, Artificial Sequence; identical to SEQ ID NO: 145
  engineered tracrRNA(mature form, having modified second region)

SEQ ID NO: 404 - RNA, 134 nt, Artificial Sequence; identical to SEQ ID NO: 147
  engineered tracrRNA(mature form, having modified second region)

SEQ ID NO: 405 - RNA, 136 nt, Artificial Sequence; identical to SEQ ID NO: 148
  engineered tracrRNA(mature form, having modified second region)

SEQ ID NO: 406 - RNA, 138 nt, Artificial Sequence; identical to SEQ ID NO: 149
  engineered tracrRNA(mature form, having modified second region)

SEQ ID NO: 407 - RNA, 110 nt, Artificial Sequence
  engineered scaffold(mature form, the second region is deleted)
cuucacugauaaaguggagaagcugcuugcaucagccuaaugucgagaagugcuuucuucggaaaguaacccucgaaacaaauucauuugaaagaaugaaggaaugcaac

SEQ ID NO: 408 - RNA, 111 nt, Artificial Sequence
  engineered scaffold(mature form, having modified second region)
cuucacugauaaaguggagaaggcugcuugcaucagccuaaugucgagaagugcuuucuucggaaaguaacccucgaaacaaauucauuugaaagaaugaaggaaugcaac

SEQ ID NO: 409 - RNA, 115 nt, Artificial Sequence
  engineered scaffold(mature form, having modified second region)
cuucacugauaaaguggagaauuagggcugcuugcaucagccuaaugucgagaagugcuuucuucggaaaguaacccucgaaacaaauucauuugaaagaaugaaggaaugcaac

SEQ ID NO: 410 - RNA, 117 nt, Artificial Sequence
  engineered scaffold(mature form, having modified second region)
cuucacugauaaaguggagaacuuaggggcugcuugcaucagccuaaugucgagaagugcuuucuucggaaaguaacccucgaaacaaauucauuugaaagaaugaaggaaugcaac

SEQ ID NO: 411 - RNA, 118 nt, Artificial Sequence
  engineered scaffold(mature form, having modified second region)
cuucacugauaaaguggagaacuuagugggcugcuugcaucagccuaaugucgagaagugcuuucuucggaaaguaacccucgaaacaaauucauuugaaagaaugaaggaaugcaac

SEQ ID NO: 412 - RNA, 120 nt, Artificial Sequence
  engineered scaffold(mature form, having modified second region)
cuucacugauaaaguggagaaccuuaggugggcugcuugcaucagccuaaugucgagaagugcuuucuucggaaaguaacccucgaaacaaauucauuugaaagaaugaaggaaugcaac

SEQ ID NO: 413 - RNA, 121 nt, Artificial Sequence
  engineered scaffold(mature form, having modified second region)
cuucacugauaaaguggagaaccguuaggugggcugcuugcaucagccuaaugucgagaagugcuuucuucggaaaguaacccucgaaacaaauucauuugaaagaaugaaggaaugcaac

SEQ ID NO: 414 - RNA, 123 nt, Artificial Sequence
  engineered scaffold(mature form, having modified second region)
cuucacugauaaaguggagaaccgcuuagggugggcugcuugcaucagccuaaugucgagaagugcuuucuucggaaaguaacccucgaaacaaauucauuugaaagaaugaaggaaugcaac

SEQ ID NO: 415 - RNA, 125 nt, Artificial Sequence
  engineered scaffold(mature form, having modified second region)
cuucacugauaaaguggagaaccgcuuuagaggugggcugcuugcaucagccuaaugucgagaagugcuuucuucggaaaguaacccucgaaacaaauucauuugaaagaaugaaggaaugcaac

SEQ ID NO: 416 - RNA, 127 nt, Artificial Sequence
  engineered scaffold(mature form, having modified second region)
cuucacugauaaaguggagaaccgcuuuuagaaggugggcugcuugcaucagccuaaugucgagaagugcuuucuucggaaaguaacccucgaaacaaauucauuugaaagaaugaaggaaugcaac

SEQ ID NO: 417 - RNA, 129 nt, Artificial Sequence
  engineered scaffold(mature form, having modified second region)
cuucacugauaaaguggagaaccgcuucuuaggaaggugggcugcuugcaucagccuaaugucgagaagugcuuucuucggaaaguaacccucgaaacaaauucauuugaaagaaugaaggaaugcaac

SEQ ID NO: 418 - RNA, 131 nt, Artificial Sequence
  engineered scaffold(mature form, having modified second region)
cuucacugauaaaguggagaaccgcuucauuagugaaggugggcugcuugcaucagccuaaugucgagaagugcuuucuucggaaaguaacccucgaaacaaauucauuugaaagaaugaaggaaugcaac

SEQ ID NO: 419 - RNA, 133 nt, Artificial Sequence
  engineered scaffold(mature form, having modified second region)
cuucacugauaaaguggagaaccgcuucacuuaggugaaggugggcugcuugcaucagccuaaugucgagaagugcuuucuucggaaaguaacccucgaaacaaauucauuugaaagaaugaaggaaugcaac

SEQ ID NO: 420 - RNA, 134 nt, Artificial Sequence
  engineered scaffold(mature form, having modified second region)
cuucacugauaaaguggagaaccgcuucacuuagagugaaggugggcugcuugcaucagccuaaugucgagaagugcuuucuucggaaaguaacccucgaaacaaauucauuugaaagaaugaaggaaugcaac

SEQ ID NO: 421 - RNA, 136 nt, Artificial Sequence
  engineered scaffold(mature form, having modified second region)
cuucacugauaaaguggagaaccgcuucaccuuaggagugaaggugggcugcuugcaucagccuaaugucgagaagugcuuucuucggaaaguaacccucgaaacaaauucauuugaaagaaugaaggaaugcaac

SEQ ID NO: 422 - RNA, 138 nt, Artificial Sequence; identical to SEQ ID NO: 188
  engineered scaffold(mature form, having modified second region)

SEQ ID NO: 423 - RNA, 140 nt, Artificial Sequence; identical to SEQ ID NO: 189
  engineered scaffold(mature form, having modified second region)

SEQ ID NO: 424 - RNA, 142 nt, Artificial Sequence; identical to SEQ ID NO: 190
  engineered scaffold(mature form, having modified second region)

SEQ ID NO: 425 - RNA, 144 nt, Artificial Sequence; identical to SEQ ID NO: 191
  engineered scaffold(mature form, having modified second region)

SEQ ID NO: 426 - RNA, 146 nt, Artificial Sequence; identical to SEQ ID NO: 192
  engineered scaffold(mature form, having modified second region)

SEQ ID NO: 427 - RNA, 148 nt, Artificial Sequence; identical to SEQ ID NO: 193
  engineered scaffold(mature form, having modified second region)

SEQ ID NO: 428 - RNA, 150 nt, Artificial Sequence; identical to SEQ ID NO: 194
  engineered scaffold(mature form, having modified second region)

SEQ ID NO: 429 - RNA, 152 nt, Artificial Sequence; identical to SEQ ID NO: 195
  engineered scaffold(mature form, having modified second region)

SEQ ID NO: 430 - RNA, 153 nt, Artificial Sequence; identical to SEQ ID NO: 196
  engineered scaffold(mature form, having modified second region)

SEQ ID NO: 431 - RNA, 155 nt, Artificial Sequence; identical to SEQ ID NO: 197
  engineered scaffold(mature form, having modified second region)

SEQ ID NO: 432 - RNA, 157 nt, Artificial Sequence; identical to SEQ ID NO: 198
  engineered scaffold(mature form, having modified second region)

SEQ ID NO: 433 - RNA, 159 nt, Artificial Sequence; identical to SEQ ID NO: 199
  engineered scaffold(mature form, having modified second region)

SEQ ID NO: 434 - RNA, 55 nt, Artificial Sequence
  modified third region
gcugcuugcaucagccuaaugucgagaagugcuuucuucggaaaguaacccucga

SEQ ID NO: 435 - RNA, 53 nt, Artificial Sequence
  modified third region
gcugcuugcaucagccuaaugucgagaagugcuuuuucgaaaguaacccucga

SEQ ID NO: 436 - RNA, 51 nt, Artificial Sequence
  modified third region
gcugcuugcaucagccuaaugucgagaagugcuuuucgaaguaacccucga

SEQ ID NO: 437 - RNA, 51 nt, Artificial Sequence
  modified third region
gcugcuugcaucagccuaaugucgagaagugcucuucggaguaacccucga

SEQ ID NO: 438 - RNA, 49 nt, Artificial Sequence
  modified third region
gcugcuugcaucagccuaaugucgagaagugcuuucgaguaacccucga

SEQ ID NO: 439 - RNA, 47 nt, Artificial Sequence
  modified third region
gcugcuugcaucagccuaaugucgagaagugcuucgguaacccucga

SEQ ID NO: 440 - RNA, 45 nt, Artificial Sequence
  modified third region
gcugcuugcaucagccuaaugucgagaaguguucguaacccucga

SEQ ID NO: 441 - RNA, 43 nt, Artificial Sequence
  modified third region
gcugcuugcaucagccuaaugucgagaaguuucgaacccucga

SEQ ID NO: 442 - RNA, 41 nt, Artificial Sequence
  modified third region
gcugcuugcaucagccuaaugucgagaaguucgacccucga

SEQ ID NO: 443 - RNA, 40 nt, Artificial Sequence
  modified third region
gcugcuugcaucagccuaaugucgagaaguucgcccucga

SEQ ID NO: 444 - RNA, 39 nt, Artificial Sequence
  modified third region
gcugcuugcaucagccuaaugucgagaauucgcccucga

SEQ ID NO: 445 - RNA, 38 nt, Artificial Sequence
  modified third region
gcugcuugcaucagccuaaugucgagaauucgccucga

SEQ ID NO: 446 - RNA, 37 nt, Artificial Sequence
  modified third region
gcugcuugcaucagccuaaugucgagauucgccucga

SEQ ID NO: 447 - RNA, 35 nt, Artificial Sequence
  modified third region
gcugcuugcaucagccuaaugucgaguucgcucga

SEQ ID NO: 448 - RNA, 138 nt, Artificial Sequence
  engineered tracrRNA(mature form, having modified third region)
cuucacugauaaaguggagaaccgcuucaccaaaagcugucccuuaggggauuagaacuugagugaaggugggcugcuugcaucagccuaaugucgagaagugcuuuuucgaaaguaacccucgaaacaaauucauuu

SEQ ID NO: 449 - RNA, 136 nt, Artificial Sequence
  engineered tracrRNA(mature form, having modified third region)
cuucacugauaaaguggagaaccgcuucaccaaaagcugucccuuaggggauuagaacuugagugaaggugggcugcuugcaucagccuaaugucgagaagugcuuuucgaaguaacccucgaaacaaauucauuu

SEQ ID NO: 450 - RNA, 136 nt, Artificial Sequence
  engineered tracrRNA(mature form, having modified third region)
cuucacugauaaaguggagaaccgcuucaccaaaagcugucccuuaggggauuagaacuugagugaaggugggcugcuugcaucagccuaaugucgagaagugcucuucggaguaacccucgaaacaaauucauuu

SEQ ID NO: 451 - RNA, 134 nt, Artificial Sequence
  engineered tracrRNA(mature form, having modified third region)
cuucacugauaaaguggagaaccgcuucaccaaaagcugucccuuaggggauuagaacuugagugaaggugggcugcuugcaucagccuaaugucgagaagugcuuucgaguaacccucgaaacaaauucauuu

SEQ ID NO: 452 - RNA, 132 nt, Artificial Sequence
  engineered tracrRNA(mature form, having modified third region)
cuucacugauaaaguggagaaccgcuucaccaaaagcugucccuuaggggauuagaacuugagugaaggugggcugcuugcaucagccuaaugucgagaagugcuucgguaacccucgaaacaaauucauuu

SEQ ID NO: 453 - RNA, 130 nt, Artificial Sequence
  engineered tracrRNA(mature form, having modified third region)
cuucacugauaaaguggagaaccgcuucaccaaaagcugucccuuaggggauuagaacuugagugaaggugggcugcuugcaucagccuaaugucgagaaguguucguaacccucgaaacaaauucauuu

SEQ ID NO: 454 - RNA, 128 nt, Artificial Sequence
  engineered tracrRNA(mature form, having modified third region)
cuucacugauaaaguggagaaccgcuucaccaaaagcugucccuuaggggauuagaacuugagugaaggugggcugcuugcaucagccuaaugucgagaaguuucgaacccucgaaacaaauucauuu

SEQ ID NO: 455 - RNA, 126 nt, Artificial Sequence
  engineered tracrRNA(mature form, having modified third region)
cuucacugauaaaguggagaaccgcuucaccaaaagcugucccuuaggggauuagaacuugagugaaggugggcugcuugcaucagccuaaugucgagaaguucgacccucgaaacaaauucauuu

SEQ ID NO: 456 - RNA, 125 nt, Artificial Sequence
  engineered tracrRNA(mature form, having modified third region)
cuucacugauaaaguggagaaccgcuucaccaaaagcugucccuuaggggauuagaacuugagugaaggugggcugcuugcaucagccuaaugucgagaaguucgcccucgaaacaaauucauuu

SEQ ID NO: 457 - RNA, 124 nt, Artificial Sequence
  engineered tracrRNA(mature form, having modified third region)
cuucacugauaaaguggagaaccgcuucaccaaaagcugucccuuaggggauuagaacuugagugaaggugggcugcuugcaucagccuaaugucgagaauucgcccucgaaacaaauucauuu

SEQ ID NO: 458 - RNA, 123 nt, Artificial Sequence
  engineered tracrRNA(mature form, having modified third region)
cuucacugauaaaguggagaaccgcuucaccaaaagcugucccuuaggggauuagaacuugagugaaggugggcugcuugcaucagccuaaugucgagaauucgccucgaaacaaauucauuu

SEQ ID NO: 459 - RNA, 122 nt, Artificial Sequence
  engineered tracrRNA(mature form, having modified third region)
cuucacugauaaaguggagaaccgcuucaccaaaagcugucccuuaggggauuagaacuugagugaaggugggcugcuugcaucagccuaaugucgagauucgccucgaaacaaauucauuu

SEQ ID NO: 460 - RNA, 120 nt, Artificial Sequence
  engineered tracrRNA(mature form, having modified third region)
cuucacugauaaaguggagaaccgcuucaccaaaagcugucccuuaggggauuagaacuugagugaaggugggcugcuugcaucagccuaaugucgaguucgcucgaaacaaauucauuu

SEQ ID NO: 461 - RNA, 161 nt, Artificial Sequence; identical to SEQ ID NO: 7
  engineered scaffold(mature form, having modified third region)

SEQ ID NO: 462 - RNA, 159 nt, Artificial Sequence
  engineered scaffold(mature form, having modified third region)
cuucacugauaaaguggagaaccgcuucaccaaaagcugucccuuaggggauuagaacuugagugaaggugggcugcuugcaucagccuaaugucgagaagugcuuuuucgaaaguaacccucgaaacaaauucauuugaaagaaugaaggaaugcaac

SEQ ID NO: 463 - RNA, 157 nt, Artificial Sequence
  engineered scaffold(mature form, having modified third region)
cuucacugauaaaguggagaaccgcuucaccaaaagcugucccuuaggggauuagaacuugagugaaggugggcugcuugcaucagccuaaugucgagaagugcuuuucgaaguaacccucgaaacaaauucauuugaaagaaugaaggaaugcaac

SEQ ID NO: 464 - RNA, 157 nt, Artificial Sequence
  engineered scaffold(mature form, having modified third region)
cuucacugauaaaguggagaaccgcuucaccaaaagcugucccuuaggggauuagaacuugagugaaggugggcugcuugcaucagccuaaugucgagaagugcucuucggaguaacccucgaaacaaauucauuugaaagaaugaaggaaugcaac

SEQ ID NO: 465 - RNA, 155 nt, Artificial Sequence
  engineered scaffold(mature form, having modified third region)
cuucacugauaaaguggagaaccgcuucaccaaaagcugucccuuaggggauuagaacuugagugaaggugggcugcuugcaucagccuaaugucgagaagugcuuucgaguaacccucgaaacaaauucauuugaaagaaugaaggaaugcaac

SEQ ID NO: 466 - RNA, 153 nt, Artificial Sequence
  engineered scaffold(mature form, having modified third region)
cuucacugauaaaguggagaaccgcuucaccaaaagcugucccuuaggggauuagaacuugagugaaggugggcugcuugcaucagccuaaugucgagaagugcuucgguaacccucgaaacaaauucauuugaaagaaugaaggaaugcaac

SEQ ID NO: 467 - RNA, 151 nt, Artificial Sequence
  engineered scaffold(mature form, having modified third region)
cuucacugauaaaguggagaaccgcuucaccaaaagcugucccuuaggggauuagaacuugagugaaggugggcugcuugcaucagccuaaugucgagaaguguucguaacccucgaaacaaauucauuugaaagaaugaaggaaugcaac

SEQ ID NO: 468 - RNA, 149 nt, Artificial Sequence
  engineered scaffold(mature form, having modified third region)
cuucacugauaaaguggagaaccgcuucaccaaaagcugucccuuaggggauuagaacuugagugaaggugggcugcuugcaucagccuaaugucgagaaguuucgaacccucgaaacaaauucauuugaaagaaugaaggaaugcaac

SEQ ID NO: 469 - RNA, 147 nt, Artificial Sequence
  engineered scaffold(mature form, having modified third region)
cuucacugauaaaguggagaaccgcuucaccaaaagcugucccuuaggggauuagaacuugagugaaggugggcugcuugcaucagccuaaugucgagaaguucgacccucgaaacaaauucauuugaaagaaugaaggaaugcaac

SEQ ID NO: 470 - RNA, 146 nt, Artificial Sequence
  engineered scaffold(mature form, having modified third region)
cuucacugauaaaguggagaaccgcuucaccaaaagcugucccuuaggggauuagaacuugagugaaggugggcugcuugcaucagccuaaugucgagaaguucgcccucgaaacaaauucauuugaaagaaugaaggaaugcaac

SEQ ID NO: 471 - RNA, 145 nt, Artificial Sequence
  engineered scaffold(mature form, having modified third region)
cuucacugauaaaguggagaaccgcuucaccaaaagcugucccuuaggggauuagaacuugagugaaggugggcugcuugcaucagccuaaugucgagaauucgcccucgaaacaaauucauuugaaagaaugaaggaaugcaac

SEQ ID NO: 472 - RNA, 144 nt, Artificial Sequence
  engineered scaffold(mature form, having modified third region)
cuucacugauaaaguggagaaccgcuucaccaaaagcugucccuuaggggauuagaacuugagugaaggugggcugcuugcaucagccuaaugucgagaauucgccucgaaacaaauucauuugaaagaaugaaggaaugcaac

SEQ ID NO: 473 - RNA, 143 nt, Artificial Sequence
  engineered scaffold(mature form, having modified third region)
cuucacugauaaaguggagaaccgcuucaccaaaagcugucccuuaggggauuagaacuugagugaaggugggcugcuugcaucagccuaaugucgagauucgccucgaaacaaauucauuugaaagaaugaaggaaugcaac

SEQ ID NO: 474 - RNA, 141 nt, Artificial Sequence
  engineered scaffold(mature form, having modified third region)
cuucacugauaaaguggagaaccgcuucaccaaaagcugucccuuaggggauuagaacuugagugaaggugggcugcuugcaucagccuaaugucgaguucgcucgaaacaaauucauuugaaagaaugaaggaaugcaac

SEQ ID NO: 475 - RNA, 26 nt, Artificial Sequence
  476%intermediate sequence of modified third region
gcugcuugcaucagccuaaugucgag

SEQ ID NO: 476 - RNA, 10 nt, Artificial Sequence
  intermediate sequence of modified third region
aaguucgacc

SEQ ID NO: 477 - RNA, 12 nt, Artificial Sequence
  intermediate sequence of modified third region
aaguuucgaacc

SEQ ID NO: 478 - RNA, 14 nt, Artificial Sequence
  intermediate sequence of modified third region
aaguguucguaacc

SEQ ID NO: 479 - RNA, 16 nt, Artificial Sequence
  intermediate sequence of modified third region
aagugcuucgguaacc

SEQ ID NO: 480 - RNA, 18 nt, Artificial Sequence
  intermediate sequence of modified third region
aagugcuuucgaguaacc

SEQ ID NO: 481 - RNA, 20 nt, Artificial Sequence
  intermediate sequence of modified third region
aagugcucuucggaguaacc

SEQ ID NO: 482 - RNA, 20 nt, Artificial Sequence
  intermediate sequence of modified third region
aagugcuuuucgaaguaacc

SEQ ID NO: 483 - RNA, 22 nt, Artificial Sequence
  intermediate sequence of modified third region
aagugcuuuuucgaaaguaacc

SEQ ID NO: 484 - RNA, 24 nt, Artificial Sequence
  intermediate sequence of modified third region
aagugcuuucuucggaaaguaacc

SEQ ID NO: 485 - RNA, 10 nt, Artificial Sequence
  deleted part of modified third region, upper stream
aagugcuuuc

SEQ ID NO: 486 - RNA, 10 nt, Artificial Sequence
  deleted part of modified third region, lower stream
gaaaguaacc

SEQ ID NO: 487 - RNA, 140 nt, Artificial Sequence
  engineered scaffold(mature form, the first region is deleted)
ccgcuucaccaaaagcugucccuuaggggauuagaacuugagugaaggugggcugcuugcaucagccuaaugucgagaagugcuuucuucggaaaguaacccucgaaacaaauucauuugaaagaaugaaggaaugcaac

SEQ ID NO: 488 - RNA, 125 nt, Artificial Sequence
  Example 2.1.1
accgcuucauuaggaaggugggcugcuugcaucagccuaaugucgagaagugcuuucuucggaaaguaacccucgaaacaaagaaaggaaugcaaccacacacacagugggcuaccuuuuauuuu

SEQ ID NO: 489 - RNA, 126 nt, Artificial Sequence
  Example 2.1.2
accgcuucauuagugaaggugggcugcuugcaucagccuaaugucgagaagugcuuucuucggaaaguaacccucgaaacaaagaaaggaaugcaaccacacacacagugggcuaccuuuuauuuu

SEQ ID NO: 490 - RNA, 128 nt, Artificial Sequence
  Example 2.1.3
accgcuucacuuaggugaaggugggcugcuugcaucagccuaaugucgagaagugcuuucuucggaaaguaacccucgaaacaaagaaaggaaugcaaccacacacacagugggcuaccuuuuauuuu

SEQ ID NO: 491 - RNA, 129 nt, Artificial Sequence
  Example 2.1.4
accgcuucacuuagagugaaggugggcugcuugcaucagccuaaugucgagaagugcuuucuucggaaaguaacccucgaaacaaagaaaggaaugcaaccacacacacagugggcuaccuuuuauuuu

SEQ ID NO: 492 - RNA, 131 nt, Artificial Sequence
  Example 2.1.5
accgcuucaccuuaggagugaaggugggcugcuugcaucagccuaaugucgagaagugcuuucuucggaaaguaacccucgaaacaaagaaaggaaugcaaccacacacacagugggcuaccuuuuauuuu

SEQ ID NO: 493 - RNA, 135 nt, Artificial Sequence
  Example 2.1.6
accgcuucaccaauuaguugagugaaggugggcugcuugcaucagccuaaugucgagaagugcuuucuucggaaaguaacccucgaaacaaagaaaggaaugcaaccacacacacagugggcuaccuuuuauuuu

SEQ ID NO: 494 - RNA, 137 nt, Artificial Sequence
  Example 2.1.7
accgcuucaccaaauuagcuugagugaaggugggcugcuugcaucagccuaaugucgagaagugcuuucuucggaaaguaacccucgaaacaaagaaaggaaugcaaccacacacacagugggcuaccuuuuauuuu

SEQ ID NO: 495 - RNA, 139 nt, Artificial Sequence
  Example 2.1.8
accgcuucaccaaaauuagacuugagugaaggugggcugcuugcaucagccuaaugucgagaagugcuuucuucggaaaguaacccucgaaacaaagaaaggaaugcaaccacacacacagugggcuaccuuuuauuuu

SEQ ID NO: 496 - RNA, 141 nt, Artificial Sequence
  Example 2.1.9
accgcuucaccaaaaguuagaacuugagugaaggugggcugcuugcaucagccuaaugucgagaagugcuuucuucggaaaguaacccucgaaacaaagaaaggaaugcaaccacacacacagugggcuaccuuuuauuuu

SEQ ID NO: 497 - RNA, 143 nt, Artificial Sequence
  Example 2.1.10
accgcuucaccaaaagcuuaggaacuugagugaaggugggcugcuugcaucagccuaaugucgagaagugcuuucuucggaaaguaacccucgaaacaaagaaaggaaugcaaccacacacacagugggcuaccuuuuauuuu

SEQ ID NO: 498 - RNA, 145 nt, Artificial Sequence
  Example 2.1.11
accgcuucaccaaaagcuuuagagaacuugagugaaggugggcugcuugcaucagccuaaugucgagaagugcuuucuucggaaaguaacccucgaaacaaagaaaggaaugcaaccacacacacagugggcuaccuuuuauuuu

SEQ ID NO: 499 - RNA, 147 nt, Artificial Sequence
  Example 2.1.12
accgcuucaccaaaagcuuuaguuagaacuugagugaaggugggcugcuugcaucagccuaaugucgagaagugcuuucuucggaaaguaacccucgaaacaaagaaaggaaugcaaccacacacacagugggcuaccuuuuauuuu

SEQ ID NO: 500 - RNA, 150 nt, Artificial Sequence
  Example 2.1.13
accgcuucaccaaaagcuguuuagauuagaacuugagugaaggugggcugcuugcaucagccuaaugucgagaagugcuuucuucggaaaguaacccucgaaacaaagaaaggaaugcaaccacacacacagugggcuaccuuuuauuuu

SEQ ID NO: 501 - RNA, 152 nt, Artificial Sequence
  Example 2.1.14
accgcuucaccaaaagcugucuuaggauuagaacuugagugaaggugggcugcuugcaucagccuaaugucgagaagugcuuucuucggaaaguaacccucgaaacaaagaaaggaaugcaaccacacacacagugggcuaccuuuuauuuu

SEQ ID NO: 502 - RNA, 156 nt, Artificial Sequence; identical to SEQ ID NO: 306
  Example 2.1.15

SEQ ID NO: 503 - RNA, 125 nt, Artificial Sequence
  Example 2.2.1
accgcuucauuaggaaggugggcugcuugcaucagccuaaugucgagaagugcuuucuucggaaaguaacccucgaaacaaagaaaggaaugcaaccauccccaggacacacacacuuuuauuuu

SEQ ID NO: 504 - RNA, 126 nt, Artificial Sequence
  Example 2.2.2
accgcuucauuagugaaggugggcugcuugcaucagccuaaugucgagaagugcuuucuucggaaaguaacccucgaaacaaagaaaggaaugcaaccauccccaggacacacacacuuuuauuuu

SEQ ID NO: 505 - RNA, 128 nt, Artificial Sequence
  Example 2.2.3
accgcuucacuuaggugaaggugggcugcuugcaucagccuaaugucgagaagugcuuucuucggaaaguaacccucgaaacaaagaaaggaaugcaaccauccccaggacacacacacuuuuauuuu

SEQ ID NO: 506 - RNA, 129 nt, Artificial Sequence
  Example 2.2.4
accgcuucacuuagagugaaggugggcugcuugcaucagccuaaugucgagaagugcuuucuucggaaaguaacccucgaaacaaagaaaggaaugcaaccauccccaggacacacacacuuuuauuuu

SEQ ID NO: 507 - RNA, 131 nt, Artificial Sequence
  Example 2.2.5
accgcuucaccuuaggagugaaggugggcugcuugcaucagccuaaugucgagaagugcuuucuucggaaaguaacccucgaaacaaagaaaggaaugcaaccauccccaggacacacacacuuuuauuuu

SEQ ID NO: 508 - RNA, 135 nt, Artificial Sequence
  Example 2.2.6
accgcuucaccaauuaguugagugaaggugggcugcuugcaucagccuaaugucgagaagugcuuucuucggaaaguaacccucgaaacaaagaaaggaaugcaaccauccccaggacacacacacuuuuauuuu

SEQ ID NO: 509 - RNA, 137 nt, Artificial Sequence
  Example 2.2.7
accgcuucaccaaauuagcuugagugaaggugggcugcuugcaucagccuaaugucgagaagugcuuucuucggaaaguaacccucgaaacaaagaaaggaaugcaaccauccccaggacacacacacuuuuauuuu

SEQ ID NO: 510 - RNA, 139 nt, Artificial Sequence
  Example 2.2.8
accgcuucaccaaaauuagacuugagugaaggugggcugcuugcaucagccuaaugucgagaagugcuuucuucggaaaguaacccucgaaacaaagaaaggaaugcaaccauccccaggacacacacacuuuuauuuu

SEQ ID NO: 511 - RNA, 141 nt, Artificial Sequence
  Example 2.2.9
accgcuucaccaaaaguuagaacuugagugaaggugggcugcuugcaucagccuaaugucgagaagugcuuucuucggaaaguaacccucgaaacaaagaaaggaaugcaaccauccccaggacacacacacuuuuauuuu

SEQ ID NO: 512 - RNA, 143 nt, Artificial Sequence
  Example 2.2.10
accgcuucaccaaaagcuuaggaacuugagugaaggugggcugcuugcaucagccuaaugucgagaagugcuuucuucggaaaguaacccucgaaacaaagaaaggaaugcaaccauccccaggacacacacacuuuuauuuu

SEQ ID NO: 513 - RNA, 145 nt, Artificial Sequence
  Example 2.2.11
accgcuucaccaaaagcuuuagagaacuugagugaaggugggcugcuugcaucagccuaaugucgagaagugcuuucuucggaaaguaacccucgaaacaaagaaaggaaugcaaccauccccaggacacacacacuuuuauuuu

SEQ ID NO: 514 - RNA, 147 nt, Artificial Sequence
  Example 2.2.12
accgcuucaccaaaagcuuuaguuagaacuugagugaaggugggcugcuugcaucagccuaaugucgagaagugcuuucuucggaaaguaacccucgaaacaaagaaaggaaugcaaccauccccaggacacacacacuuuuauuuu

SEQ ID NO: 515 - RNA, 150 nt, Artificial Sequence
  Example 2.2.13
accgcuucaccaaaagcuguuuagauuagaacuugagugaaggugggcugcuugcaucagccuaaugucgagaagugcuuucuucggaaaguaacccucgaaacaaagaaaggaaugcaaccauccccaggacacacacacuuuuauuuu

SEQ ID NO: 516 - RNA, 152 nt, Artificial Sequence
  Example 2.2.14
accgcuucaccaaaagcugucuuaggauuagaacuugagugaaggugggcugcuugcaucagccuaaugucgagaagugcuuucuucggaaaguaacccucgaaacaaagaaaggaaugcaaccauccccaggacacacacacuuuuauuuu

SEQ ID NO: 517 - RNA, 156 nt, Artificial Sequence; identical to SEQ ID NO: 321
  Example 2.2.15

SEQ ID NO: 518 - RNA, 122 nt, Artificial Sequence
  Example 3.1.1
accgcuuuuagaaggugggcugcuugcaucagccuaaugucgagaagugcuuucuucggaaaguaacccucgaaacaaagaaaggaaugcaaccacacacacagugggcuaccuuuuauuuu

SEQ ID NO: 519 - RNA, 120 nt, Artificial Sequence
  Example 3.1.2
accgcuuuagaggugggcugcuugcaucagccuaaugucgagaagugcuuucuucggaaaguaacccucgaaacaaagaaaggaaugcaaccacacacacagugggcuaccuuuuauuuu

SEQ ID NO: 520 - RNA, 119 nt, Artificial Sequence
  Example 3.1.3
accgcuuaguggugggcugcuugcaucagccuaaugucgagaagugcuuucuucggaaaguaacccucgaaacaaagaaaggaaugcaaccacacacacagugggcuaccuuuuauuuu

SEQ ID NO: 521 - RNA, 116 nt, Artificial Sequence
  Example 3.1.4
accguuaggugggcugcuugcaucagccuaaugucgagaagugcuuucuucggaaaguaacccucgaaacaaagaaaggaaugcaaccacacacacagugggcuaccuuuuauuuu

SEQ ID NO: 522 - RNA, 115 nt, Artificial Sequence
  Example 3.1.5
accuuaggugggcugcuugcaucagccuaaugucgagaagugcuuucuucggaaaguaacccucgaaacaaagaaaggaaugcaaccacacacacagugggcuaccuuuuauuuu

SEQ ID NO: 523 - RNA, 113 nt, Artificial Sequence
  Example 3.1.6
acuuagugggcugcuugcaucagccuaaugucgagaagugcuuucuucggaaaguaacccucgaaacaaagaaaggaaugcaaccacacacacagugggcuaccuuuuauuuu

SEQ ID NO: 524 - RNA, 112 nt, Artificial Sequence
  Example 3.1.7
acuuaggggcugcuugcaucagccuaaugucgagaagugcuuucuucggaaaguaacccucgaaacaaagaaaggaaugcaaccacacacacagugggcuaccuuuuauuuu

SEQ ID NO: 525 - RNA, 110 nt, Artificial Sequence
  Example 3.1.8
auuagggcugcuugcaucagccuaaugucgagaagugcuuucuucggaaaguaacccucgaaacaaagaaaggaaugcaaccacacacacagugggcuaccuuuuauuuu

SEQ ID NO: 526 - RNA, 106 nt, Artificial Sequence
  Example 3.1.9
aggcugcuugcaucagccuaaugucgagaagugcuuucuucggaaaguaacccucgaaacaaagaaaggaaugcaaccacacacacagugggcuaccuuuuauuuu

SEQ ID NO: 527 - RNA, 104 nt, Artificial Sequence
  Example 3.1.10
gcugcuugcaucagccuaaugucgagaagugcuuucuucggaaaguaacccucgaaacaaagaaaggaaugcaaccacacacacagugggcuaccuuuuauuuu

SEQ ID NO: 528 - RNA, 129 nt, Artificial Sequence; identical to SEQ ID NO: 491
  Example 3.1.11

SEQ ID NO: 529 - RNA, 156 nt, Artificial Sequence; identical to SEQ ID NO: 306
  Example 3.1.12

SEQ ID NO: 530 - RNA, 122 nt, Artificial Sequence
  Example 3.2.1
accgcuuuuagaaggugggcugcuugcaucagccuaaugucgagaagugcuuucuucggaaaguaacccucgaaacaaagaaaggaaugcaaccauccccaggacacacacacuuuuauuuu

SEQ ID NO: 531 - RNA, 120 nt, Artificial Sequence
  Example 3.2.2
accgcuuuagaggugggcugcuugcaucagccuaaugucgagaagugcuuucuucggaaaguaacccucgaaacaaagaaaggaaugcaaccauccccaggacacacacacuuuuauuuu

SEQ ID NO: 532 - RNA, 119 nt, Artificial Sequence
  Example 3.2.3
accgcuuaguggugggcugcuugcaucagccuaaugucgagaagugcuuucuucggaaaguaacccucgaaacaaagaaaggaaugcaaccauccccaggacacacacacuuuuauuuu

SEQ ID NO: 533 - RNA, 116 nt, Artificial Sequence
  Example 3.2.4
accguuaggugggcugcuugcaucagccuaaugucgagaagugcuuucuucggaaaguaacccucgaaacaaagaaaggaaugcaaccauccccaggacacacacacuuuuauuuu

SEQ ID NO: 534 - RNA, 115 nt, Artificial Sequence
  Example 3.2.5
accuuaggugggcugcuugcaucagccuaaugucgagaagugcuuucuucggaaaguaacccucgaaacaaagaaaggaaugcaaccauccccaggacacacacacuuuuauuuu

SEQ ID NO: 535 - RNA, 113 nt, Artificial Sequence
  Example 3.2.6
acuuagugggcugcuugcaucagccuaaugucgagaagugcuuucuucggaaaguaacccucgaaacaaagaaaggaaugcaaccauccccaggacacacacacuuuuauuuu

SEQ ID NO: 536 - RNA, 112 nt, Artificial Sequence
  Example 3.2.7
acuuaggggcugcuugcaucagccuaaugucgagaagugcuuucuucggaaaguaacccucgaaacaaagaaaggaaugcaaccauccccaggacacacacacuuuuauuuu

SEQ ID NO: 537 - RNA, 110 nt, Artificial Sequence
  Example 3.2.8
auuagggcugcuugcaucagccuaaugucgagaagugcuuucuucggaaaguaacccucgaaacaaagaaaggaaugcaaccauccccaggacacacacacuuuuauuuu

SEQ ID NO: 538 - RNA, 106 nt, Artificial Sequence
  Example 3.2.9
aggcugcuugcaucagccuaaugucgagaagugcuuucuucggaaaguaacccucgaaacaaagaaaggaaugcaaccauccccaggacacacacacuuuuauuuu

SEQ ID NO: 539 - RNA, 104 nt, Artificial Sequence
  Example 3.2.10
gcugcuugcaucagccuaaugucgagaagugcuuucuucggaaaguaacccucgaaacaaagaaaggaaugcaaccauccccaggacacacacacuuuuauuuu

SEQ ID NO: 540 - RNA, 129 nt, Artificial Sequence; identical to SEQ ID NO: 506
  Example 3.2.11

SEQ ID NO: 541 - RNA, 156 nt, Artificial Sequence; identical to SEQ ID NO: 321
  Example 3.2.12

SEQ ID NO: 542 - DNA, 20 bp, Artificial Sequence
  protospacer sequence for targeting FUS
gtgggtaggtccagtttggg

SEQ ID NO: 543 - DNA, 20 bp, Artificial Sequence
  protospacer sequence for targeting GAK
cagagtcccgggaacaagcc

SEQ ID NO: 544 - DNA, 20 bp, Artificial Sequence
  protospacer sequence for targeting MLH
agggaatgaaagtgaagatg

SEQ ID NO: 545 - RNA, 129 nt, Artificial Sequence
  Example 4.4.1
accgcuucaccauuagugagugaaggugggcugcuugcaucagccuaaugucgagaagugcucuucggaguaacccucgaaacaaagaaaggaaugcaacguggguagguccaguuuggguuuuauuuu

SEQ ID NO: 546 - RNA, 123 nt, Artificial Sequence
  Example 4.4.2
accgcuucaccauuagugagugaaggugggcugcuugcaucagccuaaugucgagaaguguucguaacccucgaaacaaagaaaggaaugcaacguggguagguccaguuuggguuuuauuuu

SEQ ID NO: 547 - RNA, 118 nt, Artificial Sequence
  Example 4.4.3
accgcuucaccauuagugagugaaggugggcugcuugcaucagccuaaugucgagaaguucgcccucgaaacaaagaaaggaaugcaacguggguagguccaguuuggguuuuauuuu

SEQ ID NO: 548 - RNA, 113 nt, Artificial Sequence
  Example 4.4.4
accgcuucaccauuagugagugaaggugggcugcuugcaucagccuaaugucgaguucgcucgaaacaaagaaaggaaugcaacguggguagguccaguuuggguuuuauuuu

SEQ ID NO: 549 - RNA, 129 nt, Artificial Sequence
  Example 4.5.1
accgcuucaccauuagugagugaaggugggcugcuugcaucagccuaaugucgagaagugcucuucggaguaacccucgaaacaaagaaaggaaugcaaccagagucccgggaacaagccuuuuauuuu

SEQ ID NO: 550 - RNA, 123 nt, Artificial Sequence
  Example 4.5.2
accgcuucaccauuagugagugaaggugggcugcuugcaucagccuaaugucgagaaguguucguaacccucgaaacaaagaaaggaaugcaaccagagucccgggaacaagccuuuuauuuu

SEQ ID NO: 551 - RNA, 129 nt, Artificial Sequence
  Example 4.6.1
accgcuucaccauuagugagugaaggugggcugcuugcaucagccuaaugucgagaagugcucuucggaguaacccucgaaacaaagaaaggaaugcaacagggaaugaaagugaagauguuuuauuuu

SEQ ID NO: 552 - DNA, 20 bp, Artificial Sequence
  protospacer sequence for targeting AHRR
ccttaataaagtataacttc

SEQ ID NO: 553 - DNA, 20 bp, Artificial Sequence
  protospacer sequence for targeting APEX1
aagaaggaatggtagttgag

SEQ ID NO: 554 - DNA, 20 bp, Artificial Sequence
  protospacer sequence for targeting BCL2L13
atttccaagtcaaccttatg

SEQ ID NO: 555 - DNA, 20 bp, Artificial Sequence
  protospacer sequence for targeting CARS
caacagcctcaccaggaaca

SEQ ID NO: 556 - DNA, 20 bp, Artificial Sequence
  protospacer sequence for targeting CCDC127
ggcaagggtcttgatgcatc

SEQ ID NO: 557 - DNA, 20 bp, Artificial Sequence
  protospacer sequence for targeting CLIC4
ccctggctacctcccctacc

SEQ ID NO: 558 - DNA, 20 bp, Artificial Sequence
  protospacer sequence for targeting COL8A1-1
gattcattctcagtgccatg

SEQ ID NO: 559 - DNA, 20 bp, Artificial Sequence
  protospacer sequence for targeting COL8A1-2
aggcaattgcaaccactgaa

SEQ ID NO: 560 - DNA, 20 bp, Artificial Sequence
  protospacer sequence for targeting EMX1
tactttgtcctccggttctg

SEQ ID NO: 561 - DNA, 20 bp, Artificial Sequence
  protospacer sequence for targeting FANCF-1
ggttctctctatagccattg

SEQ ID NO: 562 - DNA, 20 bp, Artificial Sequence
  protospacer sequence for targeting FANCF-2
actttagtgactagccgcca

SEQ ID NO: 563 - DNA, 20 bp, Artificial Sequence
  protospacer sequence for targeting FUS-1
gtgggtaggtccagtttggg

SEQ ID NO: 564 - DNA, 20 bp, Artificial Sequence
  protospacer sequence for targeting FUS-2
acaaagaaaccagcagtggc

SEQ ID NO: 565 - DNA, 20 bp, Artificial Sequence
  protospacer sequence for targeting GAB4
cctggtggctgagaccaggg

SEQ ID NO: 566 - DNA, 20 bp, Artificial Sequence
  protospacer sequence for targeting GAK
cagagtcccgggaacaagcc

SEQ ID NO: 567 - DNA, 20 bp, Artificial Sequence
  protospacer sequence for targeting HBB
ccaaagtgatgggccagcac

SEQ ID NO: 568 - DNA, 20 bp, Artificial Sequence
  protospacer sequence for targeting INIP
agagcagcgattgtaaggag

SEQ ID NO: 569 - DNA, 20 bp, Artificial Sequence
  protospacer sequence for targeting intergenic-01
gaaatatgactggaagtaaa

SEQ ID NO: 570 - DNA, 20 bp, Artificial Sequence
  protospacer sequence for targeting intergenic-02
cttccagtcatatttctaaa

SEQ ID NO: 571 - DNA, 20 bp, Artificial Sequence
  protospacer sequence for targeting intergenic-03
cccttattacaatcctgtgg

SEQ ID NO: 572 - DNA, 20 bp, Artificial Sequence
  protospacer sequence for targeting intergenic-04
cccccacaggattgtaataa

SEQ ID NO: 573 - DNA, 20 bp, Artificial Sequence
  protospacer sequence for targeting intergenic-05
atctccataacaatctttgg

SEQ ID NO: 574 - DNA, 20 bp, Artificial Sequence
  protospacer sequence for targeting intergenic-06
ctatccccattttacagatg

SEQ ID NO: 575 - DNA, 20 bp, Artificial Sequence
  protospacer sequence for targeting intergenic-07
ctgagatttgcgaagagtta

SEQ ID NO: 576 - DNA, 20 bp, Artificial Sequence
  protospacer sequence for targeting intergenic-08
attaaatagagtcttttgaa

SEQ ID NO: 577 - DNA, 20 bp, Artificial Sequence
  protospacer sequence for targeting intergenic-09
atattaattgcaagtttggg

SEQ ID NO: 578 - DNA, 20 bp, Artificial Sequence
  protospacer sequence for targeting intergenic-10
ggccaagtgcgaagtcagag

SEQ ID NO: 579 - DNA, 20 bp, Artificial Sequence
  protospacer sequence for targeting intergenic-11
ggggtgaacacccaagatcc

SEQ ID NO: 580 - DNA, 20 bp, Artificial Sequence
  protospacer sequence for targeting intergenic-12
gggtgggctcctggcagggc

SEQ ID NO: 581 - DNA, 20 bp, Artificial Sequence
  protospacer sequence for targeting intergenic-13
agaagcatgcaaaaccggca

SEQ ID NO: 582 - DNA, 20 bp, Artificial Sequence
  protospacer sequence for targeting intergenic-14
aagaggggaggttgactttg

SEQ ID NO: 583 - DNA, 20 bp, Artificial Sequence
  protospacer sequence for targeting intergenic-15
gtcaaataaagaaaaatacg

SEQ ID NO: 584 - DNA, 20 bp, Artificial Sequence
  protospacer sequence for targeting intergenic-16
atgcatctcagtggttaaca

SEQ ID NO: 585 - DNA, 20 bp, Artificial Sequence
  protospacer sequence for targeting intergenic-17
catacagggctctgtaccca

SEQ ID NO: 586 - DNA, 20 bp, Artificial Sequence
  protospacer sequence for targeting intergenic-18
caaagacactcaccctgttg

SEQ ID NO: 587 - DNA, 20 bp, Artificial Sequence
  protospacer sequence for targeting intergenic-19
agaacacatacccctgggcc

SEQ ID NO: 588 - DNA, 20 bp, Artificial Sequence
  protospacer sequence for targeting intergenic-20
ataataaaagtatttcctca

SEQ ID NO: 589 - DNA, 20 bp, Artificial Sequence
  protospacer sequence for targeting intergenic-21
agccgtggtcagtgagaggc

SEQ ID NO: 590 - DNA, 20 bp, Artificial Sequence
  protospacer sequence for targeting intergenic-22
gagctcattagcttggggag

SEQ ID NO: 591 - DNA, 20 bp, Artificial Sequence
  protospacer sequence for targeting intergenic-23
gaaaataactaaacttccca

SEQ ID NO: 592 - DNA, 20 bp, Artificial Sequence
  protospacer sequence for targeting intergenic-24
aattctttaagtaatttaag

SEQ ID NO: 593 - DNA, 20 bp, Artificial Sequence
  protospacer sequence for targeting intergenic-25
cttagtagtctcagaaccaa

SEQ ID NO: 594 - DNA, 20 bp, Artificial Sequence
  protospacer sequence for targeting intergenic-26
aaaggagcacaagtacaaac

SEQ ID NO: 595 - DNA, 20 bp, Artificial Sequence
  protospacer sequence for targeting intergenic-27
aatgatgcagtaatcgtgta

SEQ ID NO: 596 - DNA, 20 bp, Artificial Sequence
  protospacer sequence for targeting intergenic-28
ataaaaggaactatttacaa

SEQ ID NO: 597 - DNA, 20 bp, Artificial Sequence
  protospacer sequence for targeting KLHL29
gagagaccgctcaggctgga

SEQ ID NO: 598 - DNA, 20 bp, Artificial Sequence
  protospacer sequence for targeting LINC01551-1
attttgaagtgaccgtacga

SEQ ID NO: 599 - DNA, 20 bp, Artificial Sequence
  protospacer sequence for targeting LINC01551-2
ataatacactctttacactg

SEQ ID NO: 600 - DNA, 20 bp, Artificial Sequence
  protospacer sequence for targeting LOC100128398-1
aagagttattgtcaatagaa

SEQ ID NO: 601 - DNA, 20 bp, Artificial Sequence
  protospacer sequence for targeting LOC100128398-2
caaagaaatgtactgcctta

SEQ ID NO: 602 - DNA, 20 bp, Artificial Sequence
  protospacer sequence for targeting LOC100130876
aaataaccgtcggtttctta

SEQ ID NO: 603 - DNA, 20 bp, Artificial Sequence
  protospacer sequence for targeting LOC101926886
caaacaaaataattggctca

SEQ ID NO: 604 - DNA, 20 bp, Artificial Sequence
  protospacer sequence for targeting LOC105369597
gccatggtgaaggtgaaatc

SEQ ID NO: 605 - DNA, 20 bp, Artificial Sequence
  protospacer sequence for targeting LOC105370393-1
gcagtacacctgagggaaca

SEQ ID NO: 606 - DNA, 20 bp, Artificial Sequence
  protospacer sequence for targeting LOC105370393-2
aagaaagctacaggaaagca

SEQ ID NO: 607 - DNA, 20 bp, Artificial Sequence
  protospacer sequence for targeting LOC105374431
ctttaaaatgaggtactagg

SEQ ID NO: 608 - DNA, 20 bp, Artificial Sequence
  protospacer sequence for targeting LOC105375122
ccaaccaggtaccctgtgcc

SEQ ID NO: 609 - DNA, 20 bp, Artificial Sequence
  protospacer sequence for targeting LOC105378763
attgaaacatatacgtggta

SEQ ID NO: 610 - DNA, 20 bp, Artificial Sequence
  protospacer sequence for targeting LOC107984132
ggaaagcgcagaaaagtaaa

SEQ ID NO: 611 - DNA, 20 bp, Artificial Sequence
  protospacer sequence for targeting MLH1-1
agggaatgaaagtgaagatg

SEQ ID NO: 612 - DNA, 20 bp, Artificial Sequence
  protospacer sequence for targeting MLH1-2
gatcaatttacatcaaacta

SEQ ID NO: 613 - DNA, 20 bp, Artificial Sequence
  protospacer sequence for targeting MRPL39
atttcacaggactttgttaa

SEQ ID NO: 614 - DNA, 20 bp, Artificial Sequence
  protospacer sequence for targeting NEK10-1
agacaagctgtcttccttca

SEQ ID NO: 615 - DNA, 20 bp, Artificial Sequence
  protospacer sequence for targeting NEK10-2
atctgaagatcattgaaaca

SEQ ID NO: 616 - DNA, 20 bp, Artificial Sequence
  protospacer sequence for targeting NLGN1
gtctaatagaaatatagtac

SEQ ID NO: 617 - DNA, 20 bp, Artificial Sequence
  protospacer sequence for targeting NLRC4-1
gagggagacacaagttgata

SEQ ID NO: 618 - DNA, 20 bp, Artificial Sequence
  protospacer sequence for targeting NLRC4-2
gtctcagtcttccttgtggg

SEQ ID NO: 619 - DNA, 20 bp, Artificial Sequence
  protospacer sequence for targeting NUDT16-1
ggggtagaggtactctacag

SEQ ID NO: 620 - DNA, 20 bp, Artificial Sequence
  protospacer sequence for targeting NUDT16-2
ggggtagaggtagtctacag

SEQ ID NO: 621 - DNA, 20 bp, Artificial Sequence
  protospacer sequence for targeting OR4K17
acaagttcagaatcacctta

SEQ ID NO: 622 - DNA, 20 bp, Artificial Sequence
  protospacer sequence for targeting OSBPL5
gcattaaggccagcgctggg

SEQ ID NO: 623 - DNA, 20 bp, Artificial Sequence
  protospacer sequence for targeting P2RX5-TAX1BP3
cacataggccattcagaaac

SEQ ID NO: 624 - DNA, 20 bp, Artificial Sequence
  protospacer sequence for targeting POLRMT-1
gaaactgccccaaaaccggc

SEQ ID NO: 625 - DNA, 20 bp, Artificial Sequence
  protospacer sequence for targeting POLRMT-2
aggactatgtgtggccagtg

SEQ ID NO: 626 - DNA, 20 bp, Artificial Sequence
  protospacer sequence for targeting PWAR5
aacaaatcactgactaacca

SEQ ID NO: 627 - DNA, 20 bp, Artificial Sequence
  protospacer sequence for targeting RMST
ataatgccttttaggtgata

SEQ ID NO: 628 - DNA, 20 bp, Artificial Sequence
  protospacer sequence for targeting RPH3AL-1
attttcaaaacagccctatg

SEQ ID NO: 629 - DNA, 20 bp, Artificial Sequence
  protospacer sequence for targeting RPH3AL-2
cacaagggatctgagacttg

SEQ ID NO: 630 - DNA, 20 bp, Artificial Sequence
  protospacer sequence for targeting RSPO4-1
actcatacatcacctcctcc

SEQ ID NO: 631 - DNA, 20 bp, Artificial Sequence
  protospacer sequence for targeting RSPO4-2
aaggaaaggcttcctggagg

SEQ ID NO: 632 - DNA, 20 bp, Artificial Sequence
  protospacer sequence for targeting RSRP1-1
atataggatttagaaaccaa

SEQ ID NO: 633 - DNA, 20 bp, Artificial Sequence
  protospacer sequence for targeting RSRP1-2
gctctaatgtaagtatatcc

SEQ ID NO: 634 - DNA, 20 bp, Artificial Sequence
  protospacer sequence for targeting TYW1B
gatccgatgcaattttggga

SEQ ID NO: 635 - DNA, 20 bp, Artificial Sequence
  protospacer sequence for targeting UNCX
cctgaactcgggactcgacc

SEQ ID NO: 636 - DNA, 20 bp, Artificial Sequence
  protospacer sequence for targeting WNK1
gaacccagtgaaaaatacca

SEQ ID NO: 637 - DNA, 20 bp, Artificial Sequence
  protospacer sequence for targeting ZMYM2
gtaggctgctgttggacaga

SEQ ID NO: 638 - DNA, 20 bp, Artificial Sequence
  protospacer sequence for targeting ZNF10-1
aataagtcttaccacgtgtc

SEQ ID NO: 639 - DNA, 20 bp, Artificial Sequence
  protospacer sequence for targeting ZNF10-2
attcccacaataaccctatg

SEQ ID NO: 640 - RNA, 218 nt, Artificial Sequence
  Canonical Cas12f
cuucacugauaaaguggagaaccgcuucaccaaaagcugucccuuaggggauuagaacuugagugaaggugggcugcuugcaucagccuaaugucgagaagugcuuucuucggaaaguaacccucgaaacaaauucauuuuuccucuccaauucugcacaaguugcagaacccgaauagacgaaugaaggaaugcaacnnnnnnnnnnnnnnnnnnnn

SEQ ID NO: 641 - RNA, 218 nt, Artificial Sequence
  Canonical Cas12f targeting Intergenic22
cuucacugauaaaguggagaaccgcuucaccaaaagcugucccuuaggggauuagaacuugagugaaggugggcugcuugcaucagccuaaugucgagaagugcuuucuucggaaaguaacccucgaaacaaauucauuuuuccucuccaauucugcacaaguugcagaacccgaauagacgaaugaaggaaugcaacagaacacauaccccugggcc

SEQ ID NO: 642 - RNA, 10 nt, Artificial Sequence
  Linker variants for MF sgRNA
uucgaaagaa

SEQ ID NO: 643 - RNA, 12 nt, Artificial Sequence
  Linker variants for MF sgRNA
uucagaaaugaa

SEQ ID NO: 644 - RNA, 14 nt, Artificial Sequence
  Linker variants for MF sgRNA
uucaugaaaaugaa

SEQ ID NO: 645 - RNA, 16 nt, Artificial Sequence
  Linker variants for MF sgRNA
uucauugaaaaaugaa

SEQ ID NO: 646 - RNA, 11 nt, Artificial Sequence
  U-rich tail sequence
uuuruuuruuu

SEQ ID NO: 647 - RNA, 10 nt, Artificial Sequence
  U-rich tail sequence
uuuuruuuuu

SEQ ID NO: 648 - RNA, 11 nt, Artificial Sequence
  U-rich tail sequence
uuuuruuuuuu

SEQ ID NO: 649 - RNA, 129 nt, Artificial Sequence
  MS2/3/4/5
accgcuucacuuagagugaaggugggcugcuugcaucagccuaaugucgagaagugcuuucuucggaaaguaacccucgaaacaaagaaaggaaugcaacagaacacauaccccugggccuuuuauuuu

SEQ ID NO: 650 - DNA, 23 bp, Artificial Sequence
  Primer sequence
cggagggatcgctgtgggggtca

SEQ ID NO: 651 - DNA, 23 bp, Artificial Sequence
  Primer sequence
agtgcagatggcgaacctcgaga

SEQ ID NO: 652 - DNA, 25 bp, Artificial Sequence
  Primer sequence
cttcgagtacgcgaagaagaacaag

SEQ ID NO: 653 - DNA, 25 bp, Artificial Sequence
  Primer sequence
cttcgagtaccagaagaagaacaag

SEQ ID NO: 654 - DNA, 25 bp, Artificial Sequence
  Primer sequence
cttcgagtactggaagaagaacaag

SEQ ID NO: 655 - DNA, 25 bp, Artificial Sequence
  Primer sequence
cttcgagtacctgaagaagaacaag

SEQ ID NO: 656 - DNA, 23 bp, Artificial Sequence
  Primer sequence
ggagaacgccgcttacaacgccg

SEQ ID NO: 657 - DNA, 23 bp, Artificial Sequence
  Primer sequence
ggagaacgccctttacaacgccg

SEQ ID NO: 658 - DNA, 23 bp, Artificial Sequence
  Primer sequence
ggagaacgccgtatacaacgccg

SEQ ID NO: 659 - DNA, 19 bp, Artificial Sequence
  Primer sequence
atgatgctgggatccacgc

SEQ ID NO: 660 - DNA, 24 bp, Artificial Sequence
  Primer sequence
gttccgaccttgttcttaataaag

SEQ ID NO: 661 - DNA, 18 bp, Artificial Sequence
  Primer sequence
ttgaagtagttgttgagg

SEQ ID NO: 662 - DNA, 18 bp, Artificial Sequence
  Primer sequence
ttgaagtagttgttgagg

SEQ ID NO: 663 - DNA, 20 bp, Artificial Sequence
  Primer sequence
ttgaagtagttgttgaggtg

SEQ ID NO: 664 - DNA, 18 bp, Artificial Sequence
  Primer sequence
ttgaagtagttgttgagg

SEQ ID NO: 665 - DNA, 19 bp, Artificial Sequence
  Primer sequence
ttaaagttgcacttctcgc

SEQ ID NO: 666 - DNA, 18 bp, Artificial Sequence
  Primer sequence
ttaaagttgcacttctcg

SEQ ID NO: 667 - DNA, 19 bp, Artificial Sequence
  Primer sequence
ttaaagttgcacttctcgc

SEQ ID NO: 668 - DNA, 23 bp, Homo sapiens
cacacacacagtgggctaccatt

SEQ ID NO: 669 - DNA, 22 bp, Artificial Sequence
  Primer sequence
aagggttcgatcctctagagtc

SEQ ID NO: 670 - DNA, 18 bp, Artificial Sequence
  Primer sequence
agtggtggaggaagtggc

SEQ ID NO: 671 - DNA, 61 bp, Artificial Sequence
  Primer sequence
gatccagcctccggactctagaggatcgaacccttgccaccatggccccaaagaagaagcg

SEQ ID NO: 672 - DNA, 60 bp, Artificial Sequence
  Primer sequence
tcgcgtccatcgaccctgacccgccacttcctccaccactctttttcttttttgcctggc

SEQ ID NO: 673 - DNA, 22 bp, Artificial Sequence
  Primer sequence
aagggttcgatcctctagagtc

SEQ ID NO: 674 - DNA, 18 bp, Artificial Sequence
  Primer sequence
agtggtggaggaagtggc

SEQ ID NO: 675 - DNA, 60 bp, Artificial Sequence
  Primer sequence
gcggcggttctggtggctcaggcggcagcggccggccaccaaagaagaagcggaaggtcg

SEQ ID NO: 676 - DNA, 60 bp, Artificial Sequence
  Primer sequence
tttaaactcattactaaccggtagggatcgaaccctttcactttttcttttttgcctggc

SEQ ID NO: 677 - DNA, 22 bp, Artificial Sequence
  Primer sequence
aagggttcgatcctctagagtc

SEQ ID NO: 678 - DNA, 18 bp, Artificial Sequence
  Primer sequence
agtggtggaggaagtggc

SEQ ID NO: 679 - DNA, 61 bp, Artificial Sequence; identical to SEQ ID NO: 671
  Primer sequence

SEQ ID NO: 680 - DNA, 60 bp, Artificial Sequence; identical to SEQ ID NO: 672
  Primer sequence

SEQ ID NO: 681 - DNA, 20 bp, Artificial Sequence
  Primer sequence
ggccatggtggcaagggttc

SEQ ID NO: 682 - DNA, 21 bp, Artificial Sequence
  Primer sequence
ccaaagaagaagcggaaggtc

SEQ ID NO: 683 - DNA, 60 bp, Artificial Sequence
  Primer sequence
cctccggactctagaggatcgaacccttgccaccatggcccccaagaagaagaggaaggt

SEQ ID NO: 684 - DNA, 60 bp, Artificial Sequence
  Primer sequence
ctgggactccgtggataccgaccttccgcttcttctttggtgagactctctcagtcacgg

SEQ ID NO: 685 - DNA, 23 bp, Artificial Sequence
  Primer sequence
tagaagaattcgatccctaccgg

SEQ ID NO: 686 - DNA, 22 bp, Artificial Sequence
  Primer sequence
ctttttcttttttgcctggccg

SEQ ID NO: 687 - DNA, 74 bp, Artificial Sequence
  Primer sequence
ccaaaaggccggcggccacgaaaaaggccggccaggcaaaaaagaaaaagctcgagggcggaggcgggagcgga

SEQ ID NO: 688 - DNA, 60 bp, Artificial Sequence
  Primer sequence
tttaaactcattactaaccggtagggatcgaattcttctacacacacgcaaaatactcct

SEQ ID NO: 689 - DNA, 21 bp, Artificial Sequence
  Primer sequence
tgaaagggttcgatccctacc

SEQ ID NO: 690 - DNA, 22 bp, Artificial Sequence
  Primer sequence
tggccggccgctgccgcctgag

SEQ ID NO: 691 - DNA, 60 bp, Artificial Sequence
  Primer sequence
agcggcggttctggtggctcaggcggcagcggccggccaccaaagaagaagcggaaggtc

SEQ ID NO: 692 - DNA, 60 bp, Artificial Sequence
  Primer sequence
ttaaactcattactaaccggtagggatcgaaccctttcactttttcttttttgcctggcc

SEQ ID NO: 693 - DNA, 22 bp, Artificial Sequence
  Primer sequence
aagaattcgatccctaccggtt

SEQ ID NO: 694 - DNA, 23 bp, Artificial Sequence
  Primer sequence
ctttttcttttttgcctggccgg

SEQ ID NO: 695 - DNA, 60 bp, Artificial Sequence
  Primer sequence
ggcggccacgaaaaaggccggccaggcaaaaaagaaaaaggcggccgctggatccatggc

SEQ ID NO: 696 - DNA, 60 bp, Artificial Sequence
  Primer sequence
ccgtttaaactcattactaaccggtagggatcgaattcttttaaatctccacatcgcttt

SEQ ID NO: 697 - DNA, 23 bp, Artificial Sequence
  Primer sequence
tagaagaattcgatccctaccgg

SEQ ID NO: 698 - DNA, 22 bp, Artificial Sequence
  Primer sequence
tgaggcttccaccttccgtttc

SEQ ID NO: 699 - DNA, 80 bp, Artificial Sequence
  Primer sequence
ggaggtggttcgggtggctctggatcaagcccaaagaagaaacggaaggtggaagcctcaagaacactggttacgttcaa

SEQ ID NO: 700 - DNA, 80 bp, Artificial Sequence
  Primer sequence
gtttcagttagcctcccccgtttaaactcattactaaccggtagggatcgaattcttctataccagccaaggttcttccc

SEQ ID NO: 701 - DNA, 18 bp, Artificial Sequence
  Primer sequence
agtggtggaggaagtggc

SEQ ID NO: 702 - DNA, 22 bp, Artificial Sequence
  Primer sequence
ctttttcttttttgcctggccg

SEQ ID NO: 703 - DNA, 60 bp, Artificial Sequence
  Primer sequence
ggcggccacgaaaaaggccggccaggcaaaaaagaaaaagagtggtggaggaagtggcgg

SEQ ID NO: 704 - DNA, 60 bp, Artificial Sequence
  Primer sequence
tcgcgtccatcgaccctgacccgccacttcctccaccacttaccagccaaggttcttccc

SEQ ID NO: 705 - DNA, 22 bp, Artificial Sequence
  Primer sequence
ctttttcttttttgcctggccg

SEQ ID NO: 706 - DNA, 21 bp, Artificial Sequence
  Primer sequence
tgaaagggttcgatccctacc

SEQ ID NO: 707 - DNA, 60 bp, Artificial Sequence
  Primer sequence
ggcggccacgaaaaaggccggccaggcaaaaaagaaaaaggaagcctcagtgcaggtgaa

SEQ ID NO: 708 - DNA, 60 bp, Artificial Sequence
  Primer sequence
tttaaactcattactaaccggtagggatcgaaccctttcatgagactctctcagtcacgg

SEQ ID NO: 709 - DNA, 20 bp, Artificial Sequence
  Primer sequence
ggccatggtggcaagggttc

SEQ ID NO: 710 - DNA, 21 bp, Artificial Sequence
  Primer sequence
ccaaagaagaagcggaaggtc

SEQ ID NO: 711 - DNA, 60 bp, Artificial Sequence; identical to SEQ ID NO: 683
  Primer sequence

SEQ ID NO: 712 - DNA, 60 bp, Artificial Sequence; identical to SEQ ID NO: 684
  Primer sequence

SEQ ID NO: 713 - DNA, 23 bp, Artificial Sequence
  Primer sequence
ccaaagaagaagcggaaggtcgg

SEQ ID NO: 714 - DNA, 20 bp, Artificial Sequence
  Primer sequence
ggccatggtggcaagggttc

SEQ ID NO: 715 - DNA, 60 bp, Artificial Sequence
  Primer sequence
cctccggactctagaggatcgaacccttgccaccatggccccaaagaagaaacggaaggt

SEQ ID NO: 716 - DNA, 60 bp, Artificial Sequence; identical to SEQ ID NO: 684
  Primer sequence

SEQ ID NO: 717 - DNA, 22 bp, Artificial Sequence
  Primer sequence
tcaactttcgatggtagtcgcc

SEQ ID NO: 718 - DNA, 24 bp, Artificial Sequence
  Primer sequence
ggcctcgaaagagtcctgtattgt

SEQ ID NO: 719 - DNA, 20 bp, Artificial Sequence
  Nucleic acid encoding guide sequence
tccgttaatgtttaatcaga

SEQ ID NO: 720 - DNA, 20 bp, Artificial Sequence
  Nucleic acid encoding guide sequence
gaaacctgatcctccagtcc

SEQ ID NO: 721 - DNA, 20 bp, Artificial Sequence
  Nucleic acid encoding guide sequence
gccaggttaaggccagtgga

SEQ ID NO: 722 - DNA, 20 bp, Artificial Sequence
  Nucleic acid encoding guide sequence
atcagataggatcgtccgat

SEQ ID NO: 723 - DNA, 20 bp, Artificial Sequence
  Nucleic acid encoding guide sequence
gggagggcgaggccgaaacc

SEQ ID NO: 724 - DNA, 20 bp, Artificial Sequence
  Nucleic acid encoding guide sequence
ggagttttttcttccctctg

SEQ ID NO: 725 - DNA, 20 bp, Artificial Sequence
  Nucleic acid encoding guide sequence
gaaggctgccaggttaaggc

SEQ ID NO: 726 - DNA, 20 bp, Artificial Sequence
  Nucleic acid encoding guide sequence
tgcaccctgcacactgacct

SEQ ID NO: 727 - DNA, 20 bp, Homo sapiens
ttgcccagactggagtgcag

SEQ ID NO: 728 - DNA, 20 bp, Homo sapiens
gcccagtagatcgaggctac

SEQ ID NO: 729 - DNA, 20 bp, Homo sapiens
cctaatggtggtggcaatgg

SEQ ID NO: 730 - DNA, 21 bp, Homo sapiens
agacagggtctcactttgttg